European Patent Specification EP 4 142 775 B1, published March 25, 2026. Title: Treatment and/or prevention of a disease or a syndrome related to a virus infection. Applicant: Atlas Biotechnology S.A. The sequence listing filed with the application follows.

SEQUENCE LISTING (47 sequences)

SEQ ID NO: 1 - protein, 418 aa, Artificial Sequence
  Alpha1-Antitrypsin (AAT)
MPSSVSWGILLLAGLCCLVPVSLAEDPQGDAAQKTDTSHHDQDHPTFNKITPNLAEFAFSLYRQLAHQSNSTNIFFSPVSIATAFAMLSLGTKADTHDEILEGLNFNLTEIPEAQIHEGFQELLRTLNQPDSQLQLTTGNGLFLSEGLKLVDKFLEDVKKLYHSEAFTVNFGDTEEAKKQINDYVEKGTQGKIVDLVKELDRDTVFALVNYIFFKGKWERPFEVKDTEEEDFHVDQVTTVKVPMMKRLGMFNIQHCKKLSSWVLLMKYLGNATAIFFLPDEGKLQHLENELTHDIITKFLENEDRRSASLHLPKLSITGTYDLKSVLGQLGITKVFSNGADLSGVTEEAPLKLSKAVHKAVLTIDEKGTEAAGAMFLEAIPMSIPPEVKFNKPFVFLMIEQNTKSPLFMGKVVNPTQK

SEQ ID NO: 2 - protein, 44 aa, Artificial Sequence
  C-terminal AAT sequence 374-418
MFLEAIPMSIPPEVKFNKPFVFLMIEQNTKSPLFMGKVVNPTQK

SEQ ID NO: 3 - protein, 7 aa, Artificial Sequence
  short cyclic peptide derived from the C-terminal sequence of Alpha1-Antitrypsin
CPFVFLM

SEQ ID NO: 4 - protein, 7 aa, Artificial Sequence
  short cyclic peptide derived from the C-terminal sequence of Alpha1-Antitrypsin
CPFVFLE

SEQ ID NO: 5 - protein, 7 aa, Artificial Sequence
  short cyclic peptide derived from the C-terminal sequence of Alpha1-Antitrypsin
CPFVFLR

SEQ ID NO: 6 - protein, 7 aa, Artificial Sequence
  short cyclic peptide derived from the C-terminal sequence of Alpha1-Antitrypsin
CPEVFLM

SEQ ID NO: 7 - protein, 10 aa, Artificial Sequence
  HIV-TAT 48-57 peptide
GRKKRRQRRR

SEQ ID NO: 8 - protein, 15 aa, Artificial Sequence
  FHV-coat 35-49 peptide
RRRRNRTRRNRRRVR

SEQ ID NO: 9 - protein, 13 aa, Artificial Sequence
  HTLV-II Rex 4-16 peptide
TRRQRTRRARRNR

SEQ ID NO: 10 - protein, 19 aa, Artificial Sequence
  BMV gag 7-25 peptide
KMTRAQRRAAARRNRWTAR

SEQ ID NO: 11 - protein, 11 aa, Viruses
  Fluorogenic peptides derived from SARS-CoV spike
HTVSLLRSTSQ

SEQ ID NO: 12 - protein, 11 aa, Viruses
  Fluorogenic peptides derived from SARS-CoV-2 spike
TNSPRRARSVA

SEQ ID NO: 13 - DNA, 7394 bp, Artificial Sequence
  pCDH-CMV-MCS-EF1α-Puro lentivector
acgcgtgtagtcttatgcaatactcttgtagtcttgcaacatggtaacgatgagttagcaacatgccttacaaggagagaaaaagcaccgtgcatgccgattggtggaagtaaggtggtacgatcgtgccttattaggaaggcaacagacgggtctgacatggattggacgaaccactgaattgccgcattgcagagatattgtatttaagtgcctagctcgatacaataaacgggtctctctggttagaccagatctgagcctgggagctctctggctaactagggaacccactgcttaagcctcaataaagcttgccttgagtgcttcaagtagtgtgtgcccgtctgttgtgtgactctggtaactagagatccctcagacccttttagtcagtgtggaaaatctctagcagtggcgcccgaacagggacctgaaagcgaaagggaaaccagagctctctcgacgcaggactcggcttgctgaagcgcgcacggcaagaggcgaggggcggcgactggtgagtacgccaaaaattttgactagcggaggctagaaggagagagatgggtgcgagagcgtcagtattaagcgggggagaattagatcgcgatgggaaaaaattcggttaaggccagggggaaagaaaaaatataaattaaaacatatagtatgggcaagcagggagctagaacgattcgcagttaatcctggcctgttagaaacatcagaaggctgtagacaaatactgggacagctacaaccatcccttcagacaggatcagaagaacttagatcattatataatacagtagcaaccctctattgtgtgcatcaaaggatagagataaaagacaccaaggaagctttagacaagatagaggaagagcaaaacaaaagtaagaccaccgcacagcaagcggccactgatcttcagacctggaggaggagatatgagggacaattggagaagtgaattatataaatataaagtagtaaaaattgaaccattaggagtagcacccaccaaggcaaagagaagagtggtgcagagagaaaaaagagcagtgggaataggagctttgttccttgggttcttgggagcagcaggaagcactatgggcgcagcgtcaatgacgctgacggtacaggccagacaattattgtctggtatagtgcagcagcagaacaatttgctgagggctattgaggcgcaacagcatctgttgcaactcacagtctggggcatcaagcagctccaggcaagaatcctggctgtggaaagatacctaaaggatcaacagctcctggggatttggggttgctctggaaaactcatttgcaccactgctgtgccttggaatgctagttggagtaataaatctctggaacagatttggaatcacacgacctggatggagtgggacagagaaattaacaattacacaagcttaatacactccttaattgaagaatcgcaaaaccagcaagaaaagaatgaacaagaattattggaattagataaatgggcaagtttgtggaattggtttaacataacaaattggctgtggtatataaaattattcataatgatagtaggaggcttggtaggtttaagaatagtttttgctgtactttctatagtgaatagagttaggcagggatattcaccattatcgtttcagacccacctcccaaccccgaggggacccgacaggcccgaaggaatagaagaagaaggtggagagagagacagagacagatccattcgattagtgaacggatctcgacggtatcggttaacttttaaaagaaaaggggggattggggggtacagtgcaggggaaagaatagtagacataatagcaacagacatacaaactaaagaattacaaaaacaaattacaaaattcaaaattttatcgattactagtattatgcccagtacatgaccttatgggactttcctacttggcagtacatctacgtattagtcatcgctattaccatggtgatgcggttttggcagtacatcaatgggcgtggatagcggtttgactcacggggatttccaagtctccaccccattgacgtcaatgggagtttgttttggcaccaaaatcaacgggactttccaaaatgtcgtaacaactccgccccattgacgcaaatgggcggtaggcgtgtacggtgggaggtttatataagcagagctcgtttagtgaaccgtcagatcgcctggagacgccatccacgctgttttgacctccatagaagattctagagctagcgaattcgaatttaaatcggatccgcggccgcaaggatctgcgatcgctccggtgcccgtcagtgggcagagcgcacatcgcccacagtccccgagaagttggggggaggggtcggcaattgaacgggtgcctagagaaggtggcgcggggtaaactgggaaagtgatgtcgtgtactggctccgcctttttcccgagggtgggggagaaccgtatataagtgcagtagtcgccgtgaacgttctttttcgcaacgggtttgccgccagaacacagctgaagcttcgaggggctcgcatctctccttcacgcgcccgccgccctacctgaggccgccatccacgccggttgagtcgcgttctgccgcctcccgcctgtggtgcctcctgaactgcgtccgccgtctaggtaagtttaaagctcaggtcgagaccgggcctttgtccggcgctcccttggagcctacctagactcagccggctctccacgctttgcctgaccctgcttgctcaactctacgtctttgtttcgttttctgttctgcgccgttacagatccaagctgtgaccggcgcctacgatatgaccgagtacaagcccacggtgcgcctcgccacccgcgacgacgtccccagggccgtacgcaccctcgccgccgcgttcgccgactaccccgccacgcgccacaccgtcgatccggaccgccacatcgagcgggtcaccgagctgcaagaactcttcctcacgcgcgtcgggctcgacatcggcaaggtgtgggtcgcggacgacggcgccgcggtggcggtctggaccacgccggagagcgtcgaagcgggggcggtgttcgccgagatcggcccgcgcatggccgagttgagcggttcccggctggccgcgcagcaacagatggaaggcctcctggcgccgcaccggcccaaggagcccgcgtggttcctggccaccgtcggcgtctcgcccgaccaccagggcaagggtctgggcagcgccgtcgtgctccccggagtggaggcggccgagcgcgccggggtgcccgccttcctggagacctccgcgccccgcaacctccccttctacgagcggctcggcttcaccgtcaccgccgacgtcgaggtgcccgaaggaccgcgcacctggtgcatgacccgcaagcccggtgcctgacaatcaacctctggattacaaaatttgtgaaagattgactggtattcttaactatgttgctccttttacgctatgtggatacgctgctttaatgcctttgtatcatgctattgcttcccgtatggctttcattttctcctccttgtataaatcctggttgctgtctctttatgaggagttgtggcccgttgtcaggcaacgtggcgtggtgtgcactgtgtttgctgacgcaacccccactggttggggcattgccaccacctgtcagctcctttccgggactttcgctttccccctccctattgccacggcggaactcatcgccgcctgccttgcccgctgctggacaggggctcggctgttgggcactgacaattccgtggtgttgtcggggaaatcatcgtcctttccttggctgctcgcctgtgttgccacctggattctgcgcgggacgtccttctgctacgtcccttcggccctcaatccagcggaccttccttcccgcggcctgctgccggctctgcggcctcttccgcgtcttcgccttcgccctcagacgagtcggatctccctttgggccgcctccccgcctggtacctttaagaccaatgacttacaaggcagctgtagatcttagccactttttaaaagaaaaggggggactggaagggctaattcactcccaacgaagataagatctgctttttgcttgtactgggtctctctggttagaccagatctgagcctgggagctctctggctaactagggaacccactgcttaagcctcaataaagcttgccttgagtgcttcaagtagtgtgtgcccgtctgttgtgtgactctggtaactagagatccctcagacccttttagtcagtgtggaaaatctctagcagtagtagttcatgtcatcttattattcagtatttataacttgcaaagaaatgaatatcagagagtgagaggaacttgtttattgcagcttataatggttacaaataaagcaatagcatcacaaatttcacaaataaagcatttttttcactgcattctagttgtggtttgtccaaactcatcaatgtatcttatcatgtctggctctagctatcccgcccctaactccgcccatcccgcccctaactccgcccagttccgcccattctccgccccatggctgactaattttttttatttatgcagaggccgaggccgcctcggcctctgagctattccagaagtagtgaggaggcttttttggaggcctagacttttgcagagaccaaattcgtaatcatgtcatagctgtttcctgtgtgaaattgttatccgctcacaattccacacaacatacgagccggaagcataaagtgtaaagcctggggtgcctaatgagtgagctaactcacattaattgcgttgcgctcactgcccgctttccagtcgggaaacctgtcgtgccagctgcattaatgaatcggccaacgcgcggggagaggcggtttgcgtattgggcgctcttccgcttcctcgctcactgactcgctgcgctcggtcgttcggctgcggcgagcggtatcagctcactcaaaggcggtaatacggttatccacagaatcaggggataacgcaggaaagaacatgtgagcaaaaggccagcaaaaggccaggaaccgtaaaaaggccgcgttgctggcgtttttccataggctccgcccccctgacgagcatcacaaaaatcgacgctcaagtcagaggtggcgaaacccgacaggactataaagataccaggcgtttccccctggaagctccctcgtgcgctctcctgttccgaccctgccgcttaccggatacctgtccgcctttctcccttcgggaagcgtggcgctttctcatagctcacgctgtaggtatctcagttcggtgtaggtcgttcgctccaagctgggctgtgtgcacgaaccccccgttcagcccgaccgctgcgccttatccggtaactatcgtcttgagtccaacccggtaagacacgacttatcgccactggcagcagccactggtaacaggattagcagagcgaggtatgtaggcggtgctacagagttcttgaagtggtggcctaactacggctacactagaaggacagtatttggtatctgcgctctgctgaagccagttaccttcggaaaaagagttggtagctcttgatccggcaaacaaaccaccgctggtagcggtggtttttttgtttgcaagcagcagattacgcgcagaaaaaaaggatctcaagaagatcctttgatcttttctacggggtctgacgctcagtggaacgaaaactcacgttaagggattttggtcatgagattatcaaaaaggatcttcacctagatccttttaaattaaaaatgaagttttaaatcaatctaaagtatatatgagtaaacttggtctgacagttaccaatgcttaatcagtgaggcacctatctcagcgatctgtctatttcgttcatccatagttgcctgactccccgtcgtgtagataactacgatacgggagggcttaccatctggccccagtgctgcaatgataccgcgagacccacgctcaccggctccagatttatcagcaataaaccagccagccggaagggccgagcgcagaagtggtcctgcaactttatccgcctccatccagtctattaattgttgccgggaagctagagtaagtagttcgccagttaatagtttgcgcaacgttgttgccattgctacaggcatcgtggtgtcacgctcgtcgtttggtatggcttcattcagctccggttcccaacgatcaaggcgagttacatgatcccccatgttgtgcaaaaaagcggttagctccttcggtcctccgatcgttgtcagaagtaagttggccgcagtgttatcactcatggttatggcagcactgcataattctcttactgtcatgccatccgtaagatgcttttctgtgactggtgagtactcaaccaagtcattctgagaatagtgtatgcggcgaccgagttgctcttgcccggcgtcaatacgggataataccgcgccacatagcagaactttaaaagtgctcatcattggaaaacgttcttcggggcgaaaactctcaaggatcttaccgctgttgagatccagttcgatgtaacccactcgtgcacccaactgatcttcagcatcttttactttcaccagcgtttctgggtgagcaaaaacaggaaggcaaaatgccgcaaaaaagggaataagggcgacacggaaatgttgaatactcatactcttcctttttcaatattattgaagcatttatcagggttattgtctcatgagcggatacatatttgaatgtatttagaaaaataaacaaataggggttccgcgcacatttccccgaaaagtgccacctgacgtctaagaaaccattattatcatgacattaacctataaaaataggcgtatcacgaggccctttcgtctcgcgcgtttcggtgatgacggtgaaaacctctgacacatgcagctcccggagacggtcacagcttgtctgtaagcggatgccgggagcagacaagcccgtcagggcgcgtcagcgggtgttggcgggtgtcggggctggcttaactatgcggcatcagagcagattgtactgagagtgcaccatatgcggtgtgaaataccgcacagatgcgtaaggagaaaataccgcatcaggcgccattcgccattcaggctgcgcaactgttgggaagggcgatcggtgcgggcctcttcgctattacgccagctggcgaaagggggatgtgctgcaaggcgattaagttgggtaacgccagggttttcccagtcacgacgttgtaaaacgacggccagtgccaagctg

SEQ ID NO: 14 - DNA, 7193 bp, Artificial Sequence
  pCDH-CMV-MCS-EF1α-Blast lentivector
acgcgtgtagtcttatgcaatactcttgtagtcttgcaacatggtaacgatgagttagcaacatgccttacaaggagagaaaaagcaccgtgcatgccgattggtggaagtaaggtggtacgatcgtgccttattaggaaggcaacagacgggtctgacatggattggacgaaccactgaattgccgcattgcagagatattgtatttaagtgcctagctcgatacaataaacgggtctctctggttagaccagatctgagcctgggagctctctggctaactagggaacccactgcttaagcctcaataaagcttgccttgagtgcttcaagtagtgtgtgcccgtctgttgtgtgactctggtaactagagatccctcagacccttttagtcagtgtggaaaatctctagcagtggcgcccgaacagggacctgaaagcgaaagggaaaccagagctctctcgacgcaggactcggcttgctgaagcgcgcacggcaagaggcgaggggcggcgactggtgagtacgccaaaaattttgactagcggaggctagaaggagagagatgggtgcgagagcgtcagtattaagcgggggagaattagatcgcgatgggaaaaaattcggttaaggccagggggaaagaaaaaatataaattaaaacatatagtatgggcaagcagggagctagaacgattcgcagttaatcctggcctgttagaaacatcagaaggctgtagacaaatactgggacagctacaaccatcccttcagacaggatcagaagaacttagatcattatataatacagtagcaaccctctattgtgtgcatcaaaggatagagataaaagacaccaaggaagctttagacaagatagaggaagagcaaaacaaaagtaagaccaccgcacagcaagcggccactgatcttcagacctggaggaggagatatgagggacaattggagaagtgaattatataaatataaagtagtaaaaattgaaccattaggagtagcacccaccaaggcaaagagaagagtggtgcagagagaaaaaagagcagtgggaataggagctttgttccttgggttcttgggagcagcaggaagcactatgggcgcagcgtcaatgacgctgacggtacaggccagacaattattgtctggtatagtgcagcagcagaacaatttgctgagggctattgaggcgcaacagcatctgttgcaactcacagtctggggcatcaagcagctccaggcaagaatcctggctgtggaaagatacctaaaggatcaacagctcctggggatttggggttgctctggaaaactcatttgcaccactgctgtgccttggaatgctagttggagtaataaatctctggaacagatttggaatcacacgacctggatggagtgggacagagaaattaacaattacacaagcttaatacactccttaattgaagaatcgcaaaaccagcaagaaaagaatgaacaagaattattggaattagataaatgggcaagtttgtggaattggtttaacataacaaattggctgtggtatataaaattattcataatgatagtaggaggcttggtaggtttaagaatagtttttgctgtactttctatagtgaatagagttaggcagggatattcaccattatcgtttcagacccacctcccaaccccgaggggacccgacaggcccgaaggaatagaagaagaaggtggagagagagacagagacagatccattcgattagtgaacggatctcgacggtatcggttaacttttaaaagaaaaggggggattggggggtacagtgcaggggaaagaatagtagacataatagcaacagacatacaaactaaagaattacaaaaacaaattacaaaattcaaaattttatcgattactagtattatgcccagtacatgaccttatgggactttcctacttggcagtacatctacgtattagtcatcgctattaccatggtgatgcggttttggcagtacatcaatgggcgtggatagcggtttgactcacggggatttccaagtctccaccccattgacgtcaatgggagtttgttttggcaccaaaatcaacgggactttccaaaatgtcgtaacaactccgccccattgacgcaaatgggcggtaggcgtgtacggtgggaggtttatataagcagagctcgtttagtgaaccgtcagatcgcctggagacgccatccacgctgttttgacctccatagaagattctagagctagcgaattcgaatttaaatcggatccgcggccgcaaggatctgcgatcgctccggtgcccgtcagtgggcagagcgcacatcgcccacagtccccgagaagttggggggaggggtcggcaattgaacgggtgcctagagaaggtggcgcggggtaaactgggaaagtgatgtcgtgtactggctccgcctttttcccgagggtgggggagaaccgtatataagtgcagtagtcgccgtgaacgttctttttcgcaacgggtttgccgccagaacacagctgaagcttcgaggggctcgcatctctccttcacgcgcccgccgccctacctgaggccgccatccacgccggttgagtcgcgttctgccgcctcccgcctgtggtgcctcctgaactgcgtccgccgtctaggtaagtttaaagctcaggtcgagaccgggcctttgtccggcgctcccttggagcctacctagactcagccggctctccacgctttgcctgaccctgcttgctcaactctacgtctttgtttcgttttctgttctgcgccgttacagatccaagctgtgaccggcgcctacgatatggccaagcctttgtctcaagaagaatccaccctcattgaaagagcaacggctacaatcaacagcatccccatctctgaagactacagcgtcgccagcgcagctctctctagcgacggccgcatcttcactggtgtcaatgtatatcattttactgggggaccttgtgcagaactcgtggtgctgggcactgctgctgctgcggcagctggcaacctgacttgtatcgtcgcgatcggaaatgagaacaggggcatcttgagcccctgcggacggtgccgacaggtgcttctcgatctgcatcctgggatcaaagccatagtgaaggacagtgatggacagccgacggcagttgggattcgtgaattgctgccctctggttatgtgtgggagggctaacaatcaacctctggattacaaaatttgtgaaagattgactggtattcttaactatgttgctccttttacgctatgtggatacgctgctttaatgcctttgtatcatgctattgcttcccgtatggctttcattttctcctccttgtataaatcctggttgctgtctctttatgaggagttgtggcccgttgtcaggcaacgtggcgtggtgtgcactgtgtttgctgacgcaacccccactggttggggcattgccaccacctgtcagctcctttccgggactttcgctttccccctccctattgccacggcggaactcatcgccgcctgccttgcccgctgctggacaggggctcggctgttgggcactgacaattccgtggtgttgtcggggaaatcatcgtcctttccttggctgctcgcctgtgttgccacctggattctgcgcgggacgtccttctgctacgtcccttcggccctcaatccagcggaccttccttcccgcggcctgctgccggctctgcggcctcttccgcgtcttcgccttcgccctcagacgagtcggatctccctttgggccgcctccccgcctggtacctttaagaccaatgacttacaaggcagctgtagatcttagccactttttaaaagaaaaggggggactggaagggctaattcactcccaacgaagataagatctgctttttgcttgtactgggtctctctggttagaccagatctgagcctgggagctctctggctaactagggaacccactgcttaagcctcaataaagcttgccttgagtgcttcaagtagtgtgtgcccgtctgttgtgtgactctggtaactagagatccctcagacccttttagtcagtgtggaaaatctctagcagtagtagttcatgtcatcttattattcagtatttataacttgcaaagaaatgaatatcagagagtgagaggaacttgtttattgcagcttataatggttacaaataaagcaatagcatcacaaatttcacaaataaagcatttttttcactgcattctagttgtggtttgtccaaactcatcaatgtatcttatcatgtctggctctagctatcccgcccctaactccgcccatcccgcccctaactccgcccagttccgcccattctccgccccatggctgactaattttttttatttatgcagaggccgaggccgcctcggcctctgagctattccagaagtagtgaggaggcttttttggaggcctagacttttgcagagaccaaattcgtaatcatgtcatagctgtttcctgtgtgaaattgttatccgctcacaattccacacaacatacgagccggaagcataaagtgtaaagcctggggtgcctaatgagtgagctaactcacattaattgcgttgcgctcactgcccgctttccagtcgggaaacctgtcgtgccagctgcattaatgaatcggccaacgcgcggggagaggcggtttgcgtattgggcgctcttccgcttcctcgctcactgactcgctgcgctcggtcgttcggctgcggcgagcggtatcagctcactcaaaggcggtaatacggttatccacagaatcaggggataacgcaggaaagaacatgtgagcaaaaggccagcaaaaggccaggaaccgtaaaaaggccgcgttgctggcgtttttccataggctccgcccccctgacgagcatcacaaaaatcgacgctcaagtcagaggtggcgaaacccgacaggactataaagataccaggcgtttccccctggaagctccctcgtgcgctctcctgttccgaccctgccgcttaccggatacctgtccgcctttctcccttcgggaagcgtggcgctttctcatagctcacgctgtaggtatctcagttcggtgtaggtcgttcgctccaagctgggctgtgtgcacgaaccccccgttcagcccgaccgctgcgccttatccggtaactatcgtcttgagtccaacccggtaagacacgacttatcgccactggcagcagccactggtaacaggattagcagagcgaggtatgtaggcggtgctacagagttcttgaagtggtggcctaactacggctacactagaaggacagtatttggtatctgcgctctgctgaagccagttaccttcggaaaaagagttggtagctcttgatccggcaaacaaaccaccgctggtagcggtggtttttttgtttgcaagcagcagattacgcgcagaaaaaaaggatctcaagaagatcctttgatcttttctacggggtctgacgctcagtggaacgaaaactcacgttaagggattttggtcatgagattatcaaaaaggatcttcacctagatccttttaaattaaaaatgaagttttaaatcaatctaaagtatatatgagtaaacttggtctgacagttaccaatgcttaatcagtgaggcacctatctcagcgatctgtctatttcgttcatccatagttgcctgactccccgtcgtgtagataactacgatacgggagggcttaccatctggccccagtgctgcaatgataccgcgagacccacgctcaccggctccagatttatcagcaataaaccagccagccggaagggccgagcgcagaagtggtcctgcaactttatccgcctccatccagtctattaattgttgccgggaagctagagtaagtagttcgccagttaatagtttgcgcaacgttgttgccattgctacaggcatcgtggtgtcacgctcgtcgtttggtatggcttcattcagctccggttcccaacgatcaaggcgagttacatgatcccccatgttgtgcaaaaaagcggttagctccttcggtcctccgatcgttgtcagaagtaagttggccgcagtgttatcactcatggttatggcagcactgcataattctcttactgtcatgccatccgtaagatgcttttctgtgactggtgagtactcaaccaagtcattctgagaatagtgtatgcggcgaccgagttgctcttgcccggcgtcaatacgggataataccgcgccacatagcagaactttaaaagtgctcatcattggaaaacgttcttcggggcgaaaactctcaaggatcttaccgctgttgagatccagttcgatgtaacccactcgtgcacccaactgatcttcagcatcttttactttcaccagcgtttctgggtgagcaaaaacaggaaggcaaaatgccgcaaaaaagggaataagggcgacacggaaatgttgaatactcatactcttcctttttcaatattattgaagcatttatcagggttattgtctcatgagcggatacatatttgaatgtatttagaaaaataaacaaataggggttccgcgcacatttccccgaaaagtgccacctgacgtctaagaaaccattattatcatgacattaacctataaaaataggcgtatcacgaggccctttcgtctcgcgcgtttcggtgatgacggtgaaaacctctgacacatgcagctcccggagacggtcacagcttgtctgtaagcggatgccgggagcagacaagcccgtcagggcgcgtcagcgggtgttggcgggtgtcggggctggcttaactatgcggcatcagagcagattgtactgagagtgcaccatatgcggtgtgaaataccgcacagatgcgtaaggagaaaataccgcatcaggcgccattcgccattcaggctgcgcaactgttgggaagggcgatcggtgcgggcctcttcgctattacgccagctggcgaaagggggatgtgctgcaaggcgattaagttgggtaacgccagggttttcccagtcacgacgttgtaaaacgacggccagtgccaagctg

SEQ ID NO: 15 - DNA, 8159 bp, Artificial Sequence
  pCG1_SCoV2-S plasmid
gaattcgagctcgccccgttacataacttacggtaaatggcccgcctggctgaccgcccaacgacccccgcccattgacgtcaataatgacgtatgttcccatagtaacgccaatagggactttccattgacgtcaatgggtggagtatttacggtaaactgcccacttggcagtacatcaagtgtatcatatgccaagtacgccccctattgacgtcaatgacggtaaatggcccgcctggcattatgcccagtacatgaccttatgggactttcctacttggcagtacatctacgtattagtcatcgctattaccatggtgatgcggttttggcagtacatcaatgggcgtggatagcggtttgactcacggggatttccaagtctccaccccattgacgtcaatgggagtttgttttggcaccaaaatcaacgggactttccaaaatgtcgtaacaactccgccccattgacgcaaatgggcggtaggcgtgtacggtgggaggtctatataagcagagctcgtttagtgaaccgtcagatcgcctggagacgccatccacgctgttttgacctccatagaagacaccgggaccgatccagcctccgggggatcgatcccccgatcctgagaacttcagggtgagtttggggacccttgattgttctttctttttcgctattgtaaaattcatgttatatggagggggcaaagttttcagggtgttgtttagaatgggaagatgtcccttgtatcaccatggaccctcatgataattttgtttctttcactttctactctgttgacaaccattgtctcctcttattttcttttcattttctgtaactttttcgttaaactttagcttgcatttgtaacgaatttttaaattcacttttgtttatttgtcagattgtaagtactttctctaatcacttttttttcaaggcaatcagggtatattatattgtacttcagcacagttttagagaacaattgttataattaaatgataaggtagaatatttctgcatataaattctggctggcgtggaaatattcttattggtagaaacaactacatcctggtcatcatcctgcctttctctttatggttacaatgatatacactgtttgagatgaggataaaatactctgagtccaaaccgggcccctctgctaaccatgttcatgccttcttctttttcctacagctcctgggcaacgtgctggttattgtgctgtctcatcattttggcaaagaattgtaatacgactcactatagggcgaattcggatccgccaccatgttcgtgtttctggtgctgctgcctctggtgtccagccagtgtgtgaacctgaccacaagaacccagctgcctccagcctacaccaacagctttaccagaggcgtgtactaccccgacaaggtgttcagatccagcgtgctgcactctacccaggacctgttcctgcctttcttcagcaacgtgacctggttccacgccatccacgtgtccggcaccaatggcaccaagagattcgacaaccccgtgctgcccttcaacgacggggtgtactttgccagcaccgagaagtccaacatcatcagaggctggatcttcggcaccacactggacagcaagacccagagcctgctgatcgtgaacaacgccaccaacgtggtcatcaaagtgtgcgagttccagttctgcaacgaccccttcctgggcgtctactatcacaagaacaacaagagctggatggaaagcgagttccgggtgtacagcagcgccaacaactgcaccttcgagtacgtgtcccagcctttcctgatggacctggaaggcaagcagggcaacttcaagaacctgcgcgagttcgtgttcaagaacatcgacggctacttcaagatctacagcaagcacacccctatcaacctcgtgcgggatctgcctcagggcttctctgctctggaacccctggtggatctgcccatcggcatcaacatcacccggtttcagacactgctggccctgcacagaagctacctgacacctggcgatagcagcagcggatggacagctggtgccgccgcttactatgtgggctacctgcagcctagaaccttcctgctgaagtacaacgagaacggcaccatcaccgacgccgtggattgtgcccttgatcctctgagcgagacaaagtgcaccctgaagtccttcaccgtggaaaagggcatctaccagaccagcaacttccgggtgcagcccaccgaatccatcgtgcggttccccaatatcaccaatctgtgccccttcggcgaggtgttcaatgccaccagattcgcctctgtgtacgcctggaaccggaagcggatcagcaattgcgtggccgactactccgtgctgtacaactccgccagcttcagcaccttcaagtgctacggcgtgtcccctaccaagctgaacgacctgtgcttcacaaacgtgtacgccgacagcttcgtgatccggggagatgaagtgcggcagattgcccctggacagacaggcaagatcgccgactacaactacaagctgcccgacgacttcaccggctgtgtgattgcctggaacagcaacaacctggactccaaagtcggcggcaactacaattacctgtaccggctgttccggaagtccaatctgaagcccttcgagcgggacatctccaccgagatctatcaggccggcagcaccccttgtaacggcgtggaaggcttcaactgctacttcccactgcagtcctacggctttcagcccacaaatggcgtgggctatcagccctacagagtggtggtgctgagcttcgaactgctgcatgcccctgccacagtgtgcggccctaagaaaagcaccaatctcgtgaagaacaaatgcgtgaacttcaacttcaacggcctgaccggcaccggcgtgctgacagagagcaacaagaagttcctgccattccagcagtttggccgggatatcgccgataccacagacgccgttagagatccccagacactggaaatcctggacatcaccccttgcagcttcggcggagtgtctgtgatcacccctggcaccaacaccagcaatcaggtggcagtgctgtaccaggacgtgaactgtaccgaagtgcccgtggccattcacgccgatcagctgacacctacatggcgggtgtactccaccggcagcaatgtgtttcagaccagagccggctgtctgatcggagccgagcacgtgaacaatagctacgagtgcgacatccccatcggcgctggcatctgtgccagctaccagacacagacaaacagccccagacgggccagatctgtggccagccagagcatcattgcctacacaatgtctctgggcgccgagaacagcgtggcctactccaacaactctatcgctatccccaccaacttcaccatcagcgtgaccacagagatcctgcctgtgtccatgaccaagaccagcgtggactgcaccatgtacatctgcggcgattccaccgagtgctccaacctgctgctgcagtacggcagcttctgcacccagctgaatagagccctgacagggatcgccgtggaacaggacaagaacacccaagaggtgttcgcccaagtgaagcagatctacaagacccctcctatcaaggacttcggcggcttcaatttcagccagattctgcccgatcctagcaagcccagcaagcggagcttcatcgaggacctgctgttcaacaaagtgacactggccgacgccggcttcatcaagcagtatggcgattgtctgggcgacattgccgccagggatctgatttgcgcccagaagtttaacggactgacagtgctgccaccactgctgaccgatgagatgatcgcccagtacacatctgccctgctggccggcacaatcacaagcggctggacatttggagctggcgccgctctgcagatcccctttgctatgcagatggcctaccggttcaacggcatcggagtgacccagaatgtgctgtacgagaaccagaagctgatcgccaaccagttcaacagcgccatcggcaagatccaggacagcctgagcagcacagcaagcgccctgggaaagctgcaggacgtggtcaaccagaatgcccaggcactgaacaccctggtcaagcagctgtcctccaacttcggcgccatcagctctgtgctgaacgatatcctgagcagactggacaaggtggaagccgaggtgcagatcgacagactgatcaccggaaggctgcagtccctgcagacctacgttacccagcagctgatcagagccgccgagattagagcctctgccaatctggccgccaccaagatgtctgagtgtgtgctgggccagagcaagagagtggacttttgcggcaagggctaccacctgatgagcttccctcagtctgcccctcacggcgtggtgtttctgcacgtgacatacgtgcccgctcaagagaagaatttcaccaccgctccagccatctgccacgacggcaaagcccactttcctagagaaggcgtgttcgtgtccaacggcacccattggttcgtgacccagcggaacttctacgagccccagatcatcaccaccgacaacaccttcgtgtctggcaactgcgacgtcgtgatcggcattgtgaacaataccgtgtacgaccctctgcagcccgagctggacagcttcaaagaggaactggataagtactttaagaaccacacaagccccgacgtggacctgggcgatatcagcggaatcaatgccagcgtcgtgaacatccagaaagagatcgaccggctgaacgaggtggccaagaatctgaacgagagcctgatcgacctgcaagaactggggaagtacgagcagtacatcaagtggccctggtacatctggctgggctttatcgccggactgattgccatcgtgatggtcacaatcatgctgtgttgcatgaccagctgctgtagctgcctgaagggctgttgtagctgtggcagctgctgcaagttcgacgaggacgattctgagcccgtgctgaagggcgtgaaactgcactacacctaatctagagtcgactgtttaaacctgcaggcatgcaagctgatctttttccctctgccaaaaattatggggacatcatgaagccccttgagcatctgacttctggctaataaaggaaatttattttcattgcaatagtgtgttggaattttttgtgtctctcactcggaaggacatatgggagggcaaatcatttaaaacatcagaatgagtatttggtttagagtttggcaacatatgccatatgctggctgccatgaacaaaggtggctataaagaggtcatcagtatatgaaacagccccctgctgtccattccttattccatagaaaagccttgacttgaggttagattttttttatattttgttttgtgttatttttttctttaacatccctaaaattttccttacatgttttactagccagatttttcctcctctcctgactactcccagtcatagctgtccctcttctcttatgaactcgaggagctttttgcaaaagcctaggcctccaaaaaagcctcctcactacttctggaatagctcagaggccgaggcggcctcggcctctgcataaataaaaaaaattagtcagccatggggcggagaatgggcggaactgggcggagttaggggcgggatgggcggagttaggggcgggactatggttgctgactaattgagactgcattaatgaatcggccaacgcgcggggagaggcggtttgcgtattgggcgctcttccgcttcctcgctcactgactcgctgcgctcggtcgttcggctgcggcgagcggtatcagctcactcaaaggcggtaatacggttatccacagaatcaggggataacgcaggaaagaacatgtgagcaaaaggccagcaaaaggccaggaaccgtaaaaaggccgcgttgctggcgtttttccataggctccgcccccctgacgagcatcacaaaaatcgacgctcaagtcagaggtggcgaaacccgacaggactataaagataccaggcgtttccccctggaagctccctcgtgcgctctcctgttccgaccctgccgcttaccggatacctgtccgcctttctcccttcgggaagcgtggcgctttctcaatgctcacgctgtaggtatctcagttcggtgtaggtcgttcgctccaagctgggctgtgtgcacgaaccccccgttcagcccgaccgctgcgccttatccggtaactatcgtcttgagtccaacccggtaagacacgacttatcgccactggcagcagccactggtaacaggattagcagagcgaggtatgtaggcggtgctacagagttcttgaagtggtggcctaactacggctacactagaaggacagtatttggtatctgcgctctgctgaagccagttaccttcggaaaaagagttggtagctcttgatccggcaaacaaaccaccgctggtagcggtggtttttttgtttgcaagcagcagattacgcgcagaaaaaaaggatctcaagaagatcctttgatcttttctacggggtctgacgctcagtggaacgaaaactcacgttaagggattttggtcatgagattatcaaaaaggatcttcacctagatccttttaaattaaaaatgaagttttaaatcaatctaaagtatatatgagtaaacttggtctgacagttaccaatgcttaatcagtgaggcacctatctcagcgatctgtctatttcgttcatccatagttgcctgactccccgtcgtgtagataactacgatacgggagggcttaccatctggccccagtgctgcaatgataccgcgagacccacgctcaccggctccagatttatcagcaataaaccagccagccggaagggccgagcgcagaagtggtcctgcaactttatccgcctccatccagtctattaattgttgccgggaagctagagtaagtagttcgccagttaatagtttgcgcaacgttgttgccattgctacaggcatcgtggtgtcacgctcgtcgtttggtatggcttcattcagctccggttcccaacgatcaaggcgagttacatgatcccccatgttgtgcaaaaaagcggttagctccttcggtcctccgatcgttgtcagaagtaagttggccgcagtgttatcactcatggttatggcagcactgcataattctcttactgtcatgccatccgtaagatgcttttctgtgactggtgagtactcaaccaagtcattctgagaatagtgtatgcggcgaccgagttgctcttgcccggcgtcaatacgggataataccgcgccacatagcagaactttaaaagtgctcatcattggaaaacgttcttcggggcgaaaactctcaaggatcttaccgctgttgagatccagttcgatgtaacccactcgtgcacccaactgatcttcagcatcttttactttcaccagcgtttctgggtgagcaaaaacaggaaggcaaaatgccgcaaaaaagggaataagggcgacacggaaatgttgaatactcatactcttcctttttcaatattattgaagcatttatcagggttattgtctcatgagcggatacatatttgaatgtatttagaaaaataaacaaataggggttccgcgcacatttccccgaaaacgtcttcaagctgcctcgcgcgtttcggtgatgacggtgaaaacctctgacacatgcagctcccggagacggtcacagcttgtctgtaagcggatgccgggagcagacaagcccgtcagggcgcgtcagcgggtgttggcgggtgtcggggcgcagccatgacccagtcacgtagcgatagcggagttggcttaactatgcggcatcagagcagattgtactgagagtgcaccatatcgacgctctcccttatgcgactcctgcattaggaagcagcccagtagtaggttgaggccgttgagcaccgccgccgcaaggaatggtgctggcttatcgaaattaatcgactcactatagggagaccc

SEQ ID NO: 16 - DNA, 20 bp, Artificial Sequence
  G614 Spike primer 1
gcgtgaactgtaccgaagtg

SEQ ID NO: 17 - DNA, 17 bp, Artificial Sequence
  G614 Spike primer 2
cctggtacagcactgcc

SEQ ID NO: 18 - DNA, 18 bp, Artificial Sequence
  truncated SARS-CoV2-Spike primer 1
agcgaattcggatccgcc

SEQ ID NO: 19 - DNA, 34 bp, Artificial Sequence
  truncated SARS-CoV2-Spike primer 2
acagtcgactctagattagcagcagctgccacag

SEQ ID NO: 20 - DNA, 8159 bp, Artificial Sequence
  plasmids encoding Spike G614 Full length (FL)
gaattcgagctcgccccgttacataacttacggtaaatggcccgcctggctgaccgcccaacgacccccgcccattgacgtcaataatgacgtatgttcccatagtaacgccaatagggactttccattgacgtcaatgggtggagtatttacggtaaactgcccacttggcagtacatcaagtgtatcatatgccaagtacgccccctattgacgtcaatgacggtaaatggcccgcctggcattatgcccagtacatgaccttatgggactttcctacttggcagtacatctacgtattagtcatcgctattaccatggtgatgcggttttggcagtacatcaatgggcgtggatagcggtttgactcacggggatttccaagtctccaccccattgacgtcaatgggagtttgttttggcaccaaaatcaacgggactttccaaaatgtcgtaacaactccgccccattgacgcaaatgggcggtaggcgtgtacggtgggaggtctatataagcagagctcgtttagtgaaccgtcagatcgcctggagacgccatccacgctgttttgacctccatagaagacaccgggaccgatccagcctccgggggatcgatcccccgatcctgagaacttcagggtgagtttggggacccttgattgttctttctttttcgctattgtaaaattcatgttatatggagggggcaaagttttcagggtgttgtttagaatgggaagatgtcccttgtatcaccatggaccctcatgataattttgtttctttcactttctactctgttgacaaccattgtctcctcttattttcttttcattttctgtaactttttcgttaaactttagcttgcatttgtaacgaatttttaaattcacttttgtttatttgtcagattgtaagtactttctctaatcacttttttttcaaggcaatcagggtatattatattgtacttcagcacagttttagagaacaattgttataattaaatgataaggtagaatatttctgcatataaattctggctggcgtggaaatattcttattggtagaaacaactacatcctggtcatcatcctgcctttctctttatggttacaatgatatacactgtttgagatgaggataaaatactctgagtccaaaccgggcccctctgctaaccatgttcatgccttcttctttttcctacagctcctgggcaacgtgctggttattgtgctgtctcatcattttggcaaagaattgtaatacgactcactatagggcgaattcggatccgccaccatgttcgtgtttctggtgctgctgcctctggtgtccagccagtgtgtgaacctgaccacaagaacccagctgcctccagcctacaccaacagctttaccagaggcgtgtactaccccgacaaggtgttcagatccagcgtgctgcactctacccaggacctgttcctgcctttcttcagcaacgtgacctggttccacgccatccacgtgtccggcaccaatggcaccaagagattcgacaaccccgtgctgcccttcaacgacggggtgtactttgccagcaccgagaagtccaacatcatcagaggctggatcttcggcaccacactggacagcaagacccagagcctgctgatcgtgaacaacgccaccaacgtggtcatcaaagtgtgcgagttccagttctgcaacgaccccttcctgggcgtctactatcacaagaacaacaagagctggatggaaagcgagttccgggtgtacagcagcgccaacaactgcaccttcgagtacgtgtcccagcctttcctgatggacctggaaggcaagcagggcaacttcaagaacctgcgcgagttcgtgttcaagaacatcgacggctacttcaagatctacagcaagcacacccctatcaacctcgtgcgggatctgcctcagggcttctctgctctggaacccctggtggatctgcccatcggcatcaacatcacccggtttcagacactgctggccctgcacagaagctacctgacacctggcgatagcagcagcggatggacagctggtgccgccgcttactatgtgggctacctgcagcctagaaccttcctgctgaagtacaacgagaacggcaccatcaccgacgccgtggattgtgcccttgatcctctgagcgagacaaagtgcaccctgaagtccttcaccgtggaaaagggcatctaccagaccagcaacttccgggtgcagcccaccgaatccatcgtgcggttccccaatatcaccaatctgtgccccttcggcgaggtgttcaatgccaccagattcgcctctgtgtacgcctggaaccggaagcggatcagcaattgcgtggccgactactccgtgctgtacaactccgccagcttcagcaccttcaagtgctacggcgtgtcccctaccaagctgaacgacctgtgcttcacaaacgtgtacgccgacagcttcgtgatccggggagatgaagtgcggcagattgcccctggacagacaggcaagatcgccgactacaactacaagctgcccgacgacttcaccggctgtgtgattgcctggaacagcaacaacctggactccaaagtcggcggcaactacaattacctgtaccggctgttccggaagtccaatctgaagcccttcgagcgggacatctccaccgagatctatcaggccggcagcaccccttgtaacggcgtggaaggcttcaactgctacttcccactgcagtcctacggctttcagcccacaaatggcgtgggctatcagccctacagagtggtggtgctgagcttcgaactgctgcatgcccctgccacagtgtgcggccctaagaaaagcaccaatctcgtgaagaacaaatgcgtgaacttcaacttcaacggcctgaccggcaccggcgtgctgacagagagcaacaagaagttcctgccattccagcagtttggccgggatatcgccgataccacagacgccgttagagatccccagacactggaaatcctggacatcaccccttgcagcttcggcggagtgtctgtgatcacccctggcaccaacaccagcaatcaggtggcagtgctgtaccagggcgtgaactgtaccgaagtgcccgtggccattcacgccgatcagctgacacctacatggcgggtgtactccaccggcagcaatgtgtttcagaccagagccggctgtctgatcggagccgagcacgtgaacaatagctacgagtgcgacatccccatcggcgctggcatctgtgccagctaccagacacagacaaacagccccagacgggccagatctgtggccagccagagcatcattgcctacacaatgtctctgggcgccgagaacagcgtggcctactccaacaactctatcgctatccccaccaacttcaccatcagcgtgaccacagagatcctgcctgtgtccatgaccaagaccagcgtggactgcaccatgtacatctgcggcgattccaccgagtgctccaacctgctgctgcagtacggcagcttctgcacccagctgaatagagccctgacagggatcgccgtggaacaggacaagaacacccaagaggtgttcgcccaagtgaagcagatctacaagacccctcctatcaaggacttcggcggcttcaatttcagccagattctgcccgatcctagcaagcccagcaagcggagcttcatcgaggacctgctgttcaacaaagtgacactggccgacgccggcttcatcaagcagtatggcgattgtctgggcgacattgccgccagggatctgatttgcgcccagaagtttaacggactgacagtgctgccaccactgctgaccgatgagatgatcgcccagtacacatctgccctgctggccggcacaatcacaagcggctggacatttggagctggcgccgctctgcagatcccctttgctatgcagatggcctaccggttcaacggcatcggagtgacccagaatgtgctgtacgagaaccagaagctgatcgccaaccagttcaacagcgccatcggcaagatccaggacagcctgagcagcacagcaagcgccctgggaaagctgcaggacgtggtcaaccagaatgcccaggcactgaacaccctggtcaagcagctgtcctccaacttcggcgccatcagctctgtgctgaacgatatcctgagcagactggacaaggtggaagccgaggtgcagatcgacagactgatcaccggaaggctgcagtccctgcagacctacgttacccagcagctgatcagagccgccgagattagagcctctgccaatctggccgccaccaagatgtctgagtgtgtgctgggccagagcaagagagtggacttttgcggcaagggctaccacctgatgagcttccctcagtctgcccctcacggcgtggtgtttctgcacgtgacatacgtgcccgctcaagagaagaatttcaccaccgctccagccatctgccacgacggcaaagcccactttcctagagaaggcgtgttcgtgtccaacggcacccattggttcgtgacccagcggaacttctacgagccccagatcatcaccaccgacaacaccttcgtgtctggcaactgcgacgtcgtgatcggcattgtgaacaataccgtgtacgaccctctgcagcccgagctggacagcttcaaagaggaactggataagtactttaagaaccacacaagccccgacgtggacctgggcgatatcagcggaatcaatgccagcgtcgtgaacatccagaaagagatcgaccggctgaacgaggtggccaagaatctgaacgagagcctgatcgacctgcaagaactggggaagtacgagcagtacatcaagtggccctggtacatctggctgggctttatcgccggactgattgccatcgtgatggtcacaatcatgctgtgttgcatgaccagctgctgtagctgcctgaagggctgttgtagctgtggcagctgctgcaagttcgacgaggacgattctgagcccgtgctgaagggcgtgaaactgcactacacctaatctagagtcgactgtttaaacctgcaggcatgcaagctgatctttttccctctgccaaaaattatggggacatcatgaagccccttgagcatctgacttctggctaataaaggaaatttattttcattgcaatagtgtgttggaattttttgtgtctctcactcggaaggacatatgggagggcaaatcatttaaaacatcagaatgagtatttggtttagagtttggcaacatatgccatatgctggctgccatgaacaaaggtggctataaagaggtcatcagtatatgaaacagccccctgctgtccattccttattccatagaaaagccttgacttgaggttagattttttttatattttgttttgtgttatttttttctttaacatccctaaaattttccttacatgttttactagccagatttttcctcctctcctgactactcccagtcatagctgtccctcttctcttatgaactcgaggagctttttgcaaaagcctaggcctccaaaaaagcctcctcactacttctggaatagctcagaggccgaggcggcctcggcctctgcataaataaaaaaaattagtcagccatggggcggagaatgggcggaactgggcggagttaggggcgggatgggcggagttaggggcgggactatggttgctgactaattgagactgcattaatgaatcggccaacgcgcggggagaggcggtttgcgtattgggcgctcttccgcttcctcgctcactgactcgctgcgctcggtcgttcggctgcggcgagcggtatcagctcactcaaaggcggtaatacggttatccacagaatcaggggataacgcaggaaagaacatgtgagcaaaaggccagcaaaaggccaggaaccgtaaaaaggccgcgttgctggcgtttttccataggctccgcccccctgacgagcatcacaaaaatcgacgctcaagtcagaggtggcgaaacccgacaggactataaagataccaggcgtttccccctggaagctccctcgtgcgctctcctgttccgaccctgccgcttaccggatacctgtccgcctttctcccttcgggaagcgtggcgctttctcaatgctcacgctgtaggtatctcagttcggtgtaggtcgttcgctccaagctgggctgtgtgcacgaaccccccgttcagcccgaccgctgcgccttatccggtaactatcgtcttgagtccaacccggtaagacacgacttatcgccactggcagcagccactggtaacaggattagcagagcgaggtatgtaggcggtgctacagagttcttgaagtggtggcctaactacggctacactagaaggacagtatttggtatctgcgctctgctgaagccagttaccttcggaaaaagagttggtagctcttgatccggcaaacaaaccaccgctggtagcggtggtttttttgtttgcaagcagcagattacgcgcagaaaaaaaggatctcaagaagatcctttgatcttttctacggggtctgacgctcagtggaacgaaaactcacgttaagggattttggtcatgagattatcaaaaaggatcttcacctagatccttttaaattaaaaatgaagttttaaatcaatctaaagtatatatgagtaaacttggtctgacagttaccaatgcttaatcagtgaggcacctatctcagcgatctgtctatttcgttcatccatagttgcctgactccccgtcgtgtagataactacgatacgggagggcttaccatctggccccagtgctgcaatgataccgcgagacccacgctcaccggctccagatttatcagcaataaaccagccagccggaagggccgagcgcagaagtggtcctgcaactttatccgcctccatccagtctattaattgttgccgggaagctagagtaagtagttcgccagttaatagtttgcgcaacgttgttgccattgctacaggcatcgtggtgtcacgctcgtcgtttggtatggcttcattcagctccggttcccaacgatcaaggcgagttacatgatcccccatgttgtgcaaaaaagcggttagctccttcggtcctccgatcgttgtcagaagtaagttggccgcagtgttatcactcatggttatggcagcactgcataattctcttactgtcatgccatccgtaagatgcttttctgtgactggtgagtactcaaccaagtcattctgagaatagtgtatgcggcgaccgagttgctcttgcccggcgtcaatacgggataataccgcgccacatagcagaactttaaaagtgctcatcattggaaaacgttcttcggggcgaaaactctcaaggatcttaccgctgttgagatccagttcgatgtaacccactcgtgcacccaactgatcttcagcatcttttactttcaccagcgtttctgggtgagcaaaaacaggaaggcaaaatgccgcaaaaaagggaataagggcgacacggaaatgttgaatactcatactcttcctttttcaatattattgaagcatttatcagggttattgtctcatgagcggatacatatttgaatgtatttagaaaaataaacaaataggggttccgcgcacatttccccgaaaacgtcttcaagctgcctcgcgcgtttcggtgatgacggtgaaaacctctgacacatgcagctcccggagacggtcacagcttgtctgtaagcggatgccgggagcagacaagcccgtcagggcgcgtcagcgggtgttggcgggtgtcggggcgcagccatgacccagtcacgtagcgatagcggagttggcttaactatgcggcatcagagcagattgtactgagagtgcaccatatcgacgctctcccttatgcgactcctgcattaggaagcagcccagtagtaggttgaggccgttgagcaccgccgccgcaaggaatggtgctggcttatcgaaattaatcgactcactatagggagaccc

SEQ ID NO: 21 - DNA, 8102 bp, Artificial Sequence
  plasmids encoding Spike D614 DeltaCter
gaattcgagctcgccccgttacataacttacggtaaatggcccgcctggctgaccgcccaacgacccccgcccattgacgtcaataatgacgtatgttcccatagtaacgccaatagggactttccattgacgtcaatgggtggagtatttacggtaaactgcccacttggcagtacatcaagtgtatcatatgccaagtacgccccctattgacgtcaatgacggtaaatggcccgcctggcattatgcccagtacatgaccttatgggactttcctacttggcagtacatctacgtattagtcatcgctattaccatggtgatgcggttttggcagtacatcaatgggcgtggatagcggtttgactcacggggatttccaagtctccaccccattgacgtcaatgggagtttgttttggcaccaaaatcaacgggactttccaaaatgtcgtaacaactccgccccattgacgcaaatgggcggtaggcgtgtacggtgggaggtctatataagcagagctcgtttagtgaaccgtcagatcgcctggagacgccatccacgctgttttgacctccatagaagacaccgggaccgatccagcctccgggggatcgatcccccgatcctgagaacttcagggtgagtttggggacccttgattgttctttctttttcgctattgtaaaattcatgttatatggagggggcaaagttttcagggtgttgtttagaatgggaagatgtcccttgtatcaccatggaccctcatgataattttgtttctttcactttctactctgttgacaaccattgtctcctcttattttcttttcattttctgtaactttttcgttaaactttagcttgcatttgtaacgaatttttaaattcacttttgtttatttgtcagattgtaagtactttctctaatcacttttttttcaaggcaatcagggtatattatattgtacttcagcacagttttagagaacaattgttataattaaatgataaggtagaatatttctgcatataaattctggctggcgtggaaatattcttattggtagaaacaactacatcctggtcatcatcctgcctttctctttatggttacaatgatatacactgtttgagatgaggataaaatactctgagtccaaaccgggcccctctgctaaccatgttcatgccttcttctttttcctacagctcctgggcaacgtgctggttattgtgctgtctcatcattttggcaaagaattgtaatacgactcactatagggcgaattcggatccgccaccatgttcgtgtttctggtgctgctgcctctggtgtccagccagtgtgtgaacctgaccacaagaacccagctgcctccagcctacaccaacagctttaccagaggcgtgtactaccccgacaaggtgttcagatccagcgtgctgcactctacccaggacctgttcctgcctttcttcagcaacgtgacctggttccacgccatccacgtgtccggcaccaatggcaccaagagattcgacaaccccgtgctgcccttcaacgacggggtgtactttgccagcaccgagaagtccaacatcatcagaggctggatcttcggcaccacactggacagcaagacccagagcctgctgatcgtgaacaacgccaccaacgtggtcatcaaagtgtgcgagttccagttctgcaacgaccccttcctgggcgtctactatcacaagaacaacaagagctggatggaaagcgagttccgggtgtacagcagcgccaacaactgcaccttcgagtacgtgtcccagcctttcctgatggacctggaaggcaagcagggcaacttcaagaacctgcgcgagttcgtgttcaagaacatcgacggctacttcaagatctacagcaagcacacccctatcaacctcgtgcgggatctgcctcagggcttctctgctctggaacccctggtggatctgcccatcggcatcaacatcacccggtttcagacactgctggccctgcacagaagctacctgacacctggcgatagcagcagcggatggacagctggtgccgccgcttactatgtgggctacctgcagcctagaaccttcctgctgaagtacaacgagaacggcaccatcaccgacgccgtggattgtgcccttgatcctctgagcgagacaaagtgcaccctgaagtccttcaccgtggaaaagggcatctaccagaccagcaacttccgggtgcagcccaccgaatccatcgtgcggttccccaatatcaccaatctgtgccccttcggcgaggtgttcaatgccaccagattcgcctctgtgtacgcctggaaccggaagcggatcagcaattgcgtggccgactactccgtgctgtacaactccgccagcttcagcaccttcaagtgctacggcgtgtcccctaccaagctgaacgacctgtgcttcacaaacgtgtacgccgacagcttcgtgatccggggagatgaagtgcggcagattgcccctggacagacaggcaagatcgccgactacaactacaagctgcccgacgacttcaccggctgtgtgattgcctggaacagcaacaacctggactccaaagtcggcggcaactacaattacctgtaccggctgttccggaagtccaatctgaagcccttcgagcgggacatctccaccgagatctatcaggccggcagcaccccttgtaacggcgtggaaggcttcaactgctacttcccactgcagtcctacggctttcagcccacaaatggcgtgggctatcagccctacagagtggtggtgctgagcttcgaactgctgcatgcccctgccacagtgtgcggccctaagaaaagcaccaatctcgtgaagaacaaatgcgtgaacttcaacttcaacggcctgaccggcaccggcgtgctgacagagagcaacaagaagttcctgccattccagcagtttggccgggatatcgccgataccacagacgccgttagagatccccagacactggaaatcctggacatcaccccttgcagcttcggcggagtgtctgtgatcacccctggcaccaacaccagcaatcaggtggcagtgctgtaccaggacgtgaactgtaccgaagtgcccgtggccattcacgccgatcagctgacacctacatggcgggtgtactccaccggcagcaatgtgtttcagaccagagccggctgtctgatcggagccgagcacgtgaacaatagctacgagtgcgacatccccatcggcgctggcatctgtgccagctaccagacacagacaaacagccccagacgggccagatctgtggccagccagagcatcattgcctacacaatgtctctgggcgccgagaacagcgtggcctactccaacaactctatcgctatccccaccaacttcaccatcagcgtgaccacagagatcctgcctgtgtccatgaccaagaccagcgtggactgcaccatgtacatctgcggcgattccaccgagtgctccaacctgctgctgcagtacggcagcttctgcacccagctgaatagagccctgacagggatcgccgtggaacaggacaagaacacccaagaggtgttcgcccaagtgaagcagatctacaagacccctcctatcaaggacttcggcggcttcaatttcagccagattctgcccgatcctagcaagcccagcaagcggagcttcatcgaggacctgctgttcaacaaagtgacactggccgacgccggcttcatcaagcagtatggcgattgtctgggcgacattgccgccagggatctgatttgcgcccagaagtttaacggactgacagtgctgccaccactgctgaccgatgagatgatcgcccagtacacatctgccctgctggccggcacaatcacaagcggctggacatttggagctggcgccgctctgcagatcccctttgctatgcagatggcctaccggttcaacggcatcggagtgacccagaatgtgctgtacgagaaccagaagctgatcgccaaccagttcaacagcgccatcggcaagatccaggacagcctgagcagcacagcaagcgccctgggaaagctgcaggacgtggtcaaccagaatgcccaggcactgaacaccctggtcaagcagctgtcctccaacttcggcgccatcagctctgtgctgaacgatatcctgagcagactggacaaggtggaagccgaggtgcagatcgacagactgatcaccggaaggctgcagtccctgcagacctacgttacccagcagctgatcagagccgccgagattagagcctctgccaatctggccgccaccaagatgtctgagtgtgtgctgggccagagcaagagagtggacttttgcggcaagggctaccacctgatgagcttccctcagtctgcccctcacggcgtggtgtttctgcacgtgacatacgtgcccgctcaagagaagaatttcaccaccgctccagccatctgccacgacggcaaagcccactttcctagagaaggcgtgttcgtgtccaacggcacccattggttcgtgacccagcggaacttctacgagccccagatcatcaccaccgacaacaccttcgtgtctggcaactgcgacgtcgtgatcggcattgtgaacaataccgtgtacgaccctctgcagcccgagctggacagcttcaaagaggaactggataagtactttaagaaccacacaagccccgacgtggacctgggcgatatcagcggaatcaatgccagcgtcgtgaacatccagaaagagatcgaccggctgaacgaggtggccaagaatctgaacgagagcctgatcgacctgcaagaactggggaagtacgagcagtacatcaagtggccctggtacatctggctgggctttatcgccggactgattgccatcgtgatggtcacaatcatgctgtgttgcatgaccagctgctgtagctgcctgaagggctgttgtagctgtggcagctgctgctaatctagagtcgactgtttaaacctgcaggcatgcaagctgatctttttccctctgccaaaaattatggggacatcatgaagccccttgagcatctgacttctggctaataaaggaaatttattttcattgcaatagtgtgttggaattttttgtgtctctcactcggaaggacatatgggagggcaaatcatttaaaacatcagaatgagtatttggtttagagtttggcaacatatgccatatgctggctgccatgaacaaaggtggctataaagaggtcatcagtatatgaaacagccccctgctgtccattccttattccatagaaaagccttgacttgaggttagattttttttatattttgttttgtgttatttttttctttaacatccctaaaattttccttacatgttttactagccagatttttcctcctctcctgactactcccagtcatagctgtccctcttctcttatgaactcgaggagctttttgcaaaagcctaggcctccaaaaaagcctcctcactacttctggaatagctcagaggccgaggcggcctcggcctctgcataaataaaaaaaattagtcagccatggggcggagaatgggcggaactgggcggagttaggggcgggatgggcggagttaggggcgggactatggttgctgactaattgagactgcattaatgaatcggccaacgcgcggggagaggcggtttgcgtattgggcgctcttccgcttcctcgctcactgactcgctgcgctcggtcgttcggctgcggcgagcggtatcagctcactcaaaggcggtaatacggttatccacagaatcaggggataacgcaggaaagaacatgtgagcaaaaggccagcaaaaggccaggaaccgtaaaaaggccgcgttgctggcgtttttccataggctccgcccccctgacgagcatcacaaaaatcgacgctcaagtcagaggtggcgaaacccgacaggactataaagataccaggcgtttccccctggaagctccctcgtgcgctctcctgttccgaccctgccgcttaccggatacctgtccgcctttctcccttcgggaagcgtggcgctttctcaatgctcacgctgtaggtatctcagttcggtgtaggtcgttcgctccaagctgggctgtgtgcacgaaccccccgttcagcccgaccgctgcgccttatccggtaactatcgtcttgagtccaacccggtaagacacgacttatcgccactggcagcagccactggtaacaggattagcagagcgaggtatgtaggcggtgctacagagttcttgaagtggtggcctaactacggctacactagaaggacagtatttggtatctgcgctctgctgaagccagttaccttcggaaaaagagttggtagctcttgatccggcaaacaaaccaccgctggtagcggtggtttttttgtttgcaagcagcagattacgcgcagaaaaaaaggatctcaagaagatcctttgatcttttctacggggtctgacgctcagtggaacgaaaactcacgttaagggattttggtcatgagattatcaaaaaggatcttcacctagatccttttaaattaaaaatgaagttttaaatcaatctaaagtatatatgagtaaacttggtctgacagttaccaatgcttaatcagtgaggcacctatctcagcgatctgtctatttcgttcatccatagttgcctgactccccgtcgtgtagataactacgatacgggagggcttaccatctggccccagtgctgcaatgataccgcgagacccacgctcaccggctccagatttatcagcaataaaccagccagccggaagggccgagcgcagaagtggtcctgcaactttatccgcctccatccagtctattaattgttgccgggaagctagagtaagtagttcgccagttaatagtttgcgcaacgttgttgccattgctacaggcatcgtggtgtcacgctcgtcgtttggtatggcttcattcagctccggttcccaacgatcaaggcgagttacatgatcccccatgttgtgcaaaaaagcggttagctccttcggtcctccgatcgttgtcagaagtaagttggccgcagtgttatcactcatggttatggcagcactgcataattctcttactgtcatgccatccgtaagatgcttttctgtgactggtgagtactcaaccaagtcattctgagaatagtgtatgcggcgaccgagttgctcttgcccggcgtcaatacgggataataccgcgccacatagcagaactttaaaagtgctcatcattggaaaacgttcttcggggcgaaaactctcaaggatcttaccgctgttgagatccagttcgatgtaacccactcgtgcacccaactgatcttcagcatcttttactttcaccagcgtttctgggtgagcaaaaacaggaaggcaaaatgccgcaaaaaagggaataagggcgacacggaaatgttgaatactcatactcttcctttttcaatattattgaagcatttatcagggttattgtctcatgagcggatacatatttgaatgtatttagaaaaataaacaaataggggttccgcgcacatttccccgaaaacgtcttcaagctgcctcgcgcgtttcggtgatgacggtgaaaacctctgacacatgcagctcccggagacggtcacagcttgtctgtaagcggatgccgggagcagacaagcccgtcagggcgcgtcagcgggtgttggcgggtgtcggggcgcagccatgacccagtcacgtagcgatagcggagttggcttaactatgcggcatcagagcagattgtactgagagtgcaccatatcgacgctctcccttatgcgactcctgcattaggaagcagcccagtagtaggttgaggccgttgagcaccgccgccgcaaggaatggtgctggcttatcgaaattaatcgactcactatagggagaccc

SEQ ID NO: 22 - DNA, 8102 bp, Artificial Sequence
  plasmids Spike G614 DeltaCter
gaattcgagctcgccccgttacataacttacggtaaatggcccgcctggctgaccgcccaacgacccccgcccattgacgtcaataatgacgtatgttcccatagtaacgccaatagggactttccattgacgtcaatgggtggagtatttacggtaaactgcccacttggcagtacatcaagtgtatcatatgccaagtacgccccctattgacgtcaatgacggtaaatggcccgcctggcattatgcccagtacatgaccttatgggactttcctacttggcagtacatctacgtattagtcatcgctattaccatggtgatgcggttttggcagtacatcaatgggcgtggatagcggtttgactcacggggatttccaagtctccaccccattgacgtcaatgggagtttgttttggcaccaaaatcaacgggactttccaaaatgtcgtaacaactccgccccattgacgcaaatgggcggtaggcgtgtacggtgggaggtctatataagcagagctcgtttagtgaaccgtcagatcgcctggagacgccatccacgctgttttgacctccatagaagacaccgggaccgatccagcctccgggggatcgatcccccgatcctgagaacttcagggtgagtttggggacccttgattgttctttctttttcgctattgtaaaattcatgttatatggagggggcaaagttttcagggtgttgtttagaatgggaagatgtcccttgtatcaccatggaccctcatgataattttgtttctttcactttctactctgttgacaaccattgtctcctcttattttcttttcattttctgtaactttttcgttaaactttagcttgcatttgtaacgaatttttaaattcacttttgtttatttgtcagattgtaagtactttctctaatcacttttttttcaaggcaatcagggtatattatattgtacttcagcacagttttagagaacaattgttataattaaatgataaggtagaatatttctgcatataaattctggctggcgtggaaatattcttattggtagaaacaactacatcctggtcatcatcctgcctttctctttatggttacaatgatatacactgtttgagatgaggataaaatactctgagtccaaaccgggcccctctgctaaccatgttcatgccttcttctttttcctacagctcctgggcaacgtgctggttattgtgctgtctcatcattttggcaaagaattgtaatacgactcactatagggcgaattcggatccgccaccatgttcgtgtttctggtgctgctgcctctggtgtccagccagtgtgtgaacctgaccacaagaacccagctgcctccagcctacaccaacagctttaccagaggcgtgtactaccccgacaaggtgttcagatccagcgtgctgcactctacccaggacctgttcctgcctttcttcagcaacgtgacctggttccacgccatccacgtgtccggcaccaatggcaccaagagattcgacaaccccgtgctgcccttcaacgacggggtgtactttgccagcaccgagaagtccaacatcatcagaggctggatcttcggcaccacactggacagcaagacccagagcctgctgatcgtgaacaacgccaccaacgtggtcatcaaagtgtgcgagttccagttctgcaacgaccccttcctgggcgtctactatcacaagaacaacaagagctggatggaaagcgagttccgggtgtacagcagcgccaacaactgcaccttcgagtacgtgtcccagcctttcctgatggacctggaaggcaagcagggcaacttcaagaacctgcgcgagttcgtgttcaagaacatcgacggctacttcaagatctacagcaagcacacccctatcaacctcgtgcgggatctgcctcagggcttctctgctctggaacccctggtggatctgcccatcggcatcaacatcacccggtttcagacactgctggccctgcacagaagctacctgacacctggcgatagcagcagcggatggacagctggtgccgccgcttactatgtgggctacctgcagcctagaaccttcctgctgaagtacaacgagaacggcaccatcaccgacgccgtggattgtgcccttgatcctctgagcgagacaaagtgcaccctgaagtccttcaccgtggaaaagggcatctaccagaccagcaacttccgggtgcagcccaccgaatccatcgtgcggttccccaatatcaccaatctgtgccccttcggcgaggtgttcaatgccaccagattcgcctctgtgtacgcctggaaccggaagcggatcagcaattgcgtggccgactactccgtgctgtacaactccgccagcttcagcaccttcaagtgctacggcgtgtcccctaccaagctgaacgacctgtgcttcacaaacgtgtacgccgacagcttcgtgatccggggagatgaagtgcggcagattgcccctggacagacaggcaagatcgccgactacaactacaagctgcccgacgacttcaccggctgtgtgattgcctggaacagcaacaacctggactccaaagtcggcggcaactacaattacctgtaccggctgttccggaagtccaatctgaagcccttcgagcgggacatctccaccgagatctatcaggccggcagcaccccttgtaacggcgtggaaggcttcaactgctacttcccactgcagtcctacggctttcagcccacaaatggcgtgggctatcagccctacagagtggtggtgctgagcttcgaactgctgcatgcccctgccacagtgtgcggccctaagaaaagcaccaatctcgtgaagaacaaatgcgtgaacttcaacttcaacggcctgaccggcaccggcgtgctgacagagagcaacaagaagttcctgccattccagcagtttggccgggatatcgccgataccacagacgccgttagagatccccagacactggaaatcctggacatcaccccttgcagcttcggcggagtgtctgtgatcacccctggcaccaacaccagcaatcaggtggcagtgctgtaccagggcgtgaactgtaccgaagtgcccgtggccattcacgccgatcagctgacacctacatggcgggtgtactccaccggcagcaatgtgtttcagaccagagccggctgtctgatcggagccgagcacgtgaacaatagctacgagtgcgacatccccatcggcgctggcatctgtgccagctaccagacacagacaaacagccccagacgggccagatctgtggccagccagagcatcattgcctacacaatgtctctgggcgccgagaacagcgtggcctactccaacaactctatcgctatccccaccaacttcaccatcagcgtgaccacagagatcctgcctgtgtccatgaccaagaccagcgtggactgcaccatgtacatctgcggcgattccaccgagtgctccaacctgctgctgcagtacggcagcttctgcacccagctgaatagagccctgacagggatcgccgtggaacaggacaagaacacccaagaggtgttcgcccaagtgaagcagatctacaagacccctcctatcaaggacttcggcggcttcaatttcagccagattctgcccgatcctagcaagcccagcaagcggagcttcatcgaggacctgctgttcaacaaagtgacactggccgacgccggcttcatcaagcagtatggcgattgtctgggcgacattgccgccagggatctgatttgcgcccagaagtttaacggactgacagtgctgccaccactgctgaccgatgagatgatcgcccagtacacatctgccctgctggccggcacaatcacaagcggctggacatttggagctggcgccgctctgcagatcccctttgctatgcagatggcctaccggttcaacggcatcggagtgacccagaatgtgctgtacgagaaccagaagctgatcgccaaccagttcaacagcgccatcggcaagatccaggacagcctgagcagcacagcaagcgccctgggaaagctgcaggacgtggtcaaccagaatgcccaggcactgaacaccctggtcaagcagctgtcctccaacttcggcgccatcagctctgtgctgaacgatatcctgagcagactggacaaggtggaagccgaggtgcagatcgacagactgatcaccggaaggctgcagtccctgcagacctacgttacccagcagctgatcagagccgccgagattagagcctctgccaatctggccgccaccaagatgtctgagtgtgtgctgggccagagcaagagagtggacttttgcggcaagggctaccacctgatgagcttccctcagtctgcccctcacggcgtggtgtttctgcacgtgacatacgtgcccgctcaagagaagaatttcaccaccgctccagccatctgccacgacggcaaagcccactttcctagagaaggcgtgttcgtgtccaacggcacccattggttcgtgacccagcggaacttctacgagccccagatcatcaccaccgacaacaccttcgtgtctggcaactgcgacgtcgtgatcggcattgtgaacaataccgtgtacgaccctctgcagcccgagctggacagcttcaaagaggaactggataagtactttaagaaccacacaagccccgacgtggacctgggcgatatcagcggaatcaatgccagcgtcgtgaacatccagaaagagatcgaccggctgaacgaggtggccaagaatctgaacgagagcctgatcgacctgcaagaactggggaagtacgagcagtacatcaagtggccctggtacatctggctgggctttatcgccggactgattgccatcgtgatggtcacaatcatgctgtgttgcatgaccagctgctgtagctgcctgaagggctgttgtagctgtggcagctgctgctaatctagagtcgactgtttaaacctgcaggcatgcaagctgatctttttccctctgccaaaaattatggggacatcatgaagccccttgagcatctgacttctggctaataaaggaaatttattttcattgcaatagtgtgttggaattttttgtgtctctcactcggaaggacatatgggagggcaaatcatttaaaacatcagaatgagtatttggtttagagtttggcaacatatgccatatgctggctgccatgaacaaaggtggctataaagaggtcatcagtatatgaaacagccccctgctgtccattccttattccatagaaaagccttgacttgaggttagattttttttatattttgttttgtgttatttttttctttaacatccctaaaattttccttacatgttttactagccagatttttcctcctctcctgactactcccagtcatagctgtccctcttctcttatgaactcgaggagctttttgcaaaagcctaggcctccaaaaaagcctcctcactacttctggaatagctcagaggccgaggcggcctcggcctctgcataaataaaaaaaattagtcagccatggggcggagaatgggcggaactgggcggagttaggggcgggatgggcggagttaggggcgggactatggttgctgactaattgagactgcattaatgaatcggccaacgcgcggggagaggcggtttgcgtattgggcgctcttccgcttcctcgctcactgactcgctgcgctcggtcgttcggctgcggcgagcggtatcagctcactcaaaggcggtaatacggttatccacagaatcaggggataacgcaggaaagaacatgtgagcaaaaggccagcaaaaggccaggaaccgtaaaaaggccgcgttgctggcgtttttccataggctccgcccccctgacgagcatcacaaaaatcgacgctcaagtcagaggtggcgaaacccgacaggactataaagataccaggcgtttccccctggaagctccctcgtgcgctctcctgttccgaccctgccgcttaccggatacctgtccgcctttctcccttcgggaagcgtggcgctttctcaatgctcacgctgtaggtatctcagttcggtgtaggtcgttcgctccaagctgggctgtgtgcacgaaccccccgttcagcccgaccgctgcgccttatccggtaactatcgtcttgagtccaacccggtaagacacgacttatcgccactggcagcagccactggtaacaggattagcagagcgaggtatgtaggcggtgctacagagttcttgaagtggtggcctaactacggctacactagaaggacagtatttggtatctgcgctctgctgaagccagttaccttcggaaaaagagttggtagctcttgatccggcaaacaaaccaccgctggtagcggtggtttttttgtttgcaagcagcagattacgcgcagaaaaaaaggatctcaagaagatcctttgatcttttctacggggtctgacgctcagtggaacgaaaactcacgttaagggattttggtcatgagattatcaaaaaggatcttcacctagatccttttaaattaaaaatgaagttttaaatcaatctaaagtatatatgagtaaacttggtctgacagttaccaatgcttaatcagtgaggcacctatctcagcgatctgtctatttcgttcatccatagttgcctgactccccgtcgtgtagataactacgatacgggagggcttaccatctggccccagtgctgcaatgataccgcgagacccacgctcaccggctccagatttatcagcaataaaccagccagccggaagggccgagcgcagaagtggtcctgcaactttatccgcctccatccagtctattaattgttgccgggaagctagagtaagtagttcgccagttaatagtttgcgcaacgttgttgccattgctacaggcatcgtggtgtcacgctcgtcgtttggtatggcttcattcagctccggttcccaacgatcaaggcgagttacatgatcccccatgttgtgcaaaaaagcggttagctccttcggtcctccgatcgttgtcagaagtaagttggccgcagtgttatcactcatggttatggcagcactgcataattctcttactgtcatgccatccgtaagatgcttttctgtgactggtgagtactcaaccaagtcattctgagaatagtgtatgcggcgaccgagttgctcttgcccggcgtcaatacgggataataccgcgccacatagcagaactttaaaagtgctcatcattggaaaacgttcttcggggcgaaaactctcaaggatcttaccgctgttgagatccagttcgatgtaacccactcgtgcacccaactgatcttcagcatcttttactttcaccagcgtttctgggtgagcaaaaacaggaaggcaaaatgccgcaaaaaagggaataagggcgacacggaaatgttgaatactcatactcttcctttttcaatattattgaagcatttatcagggttattgtctcatgagcggatacatatttgaatgtatttagaaaaataaacaaataggggttccgcgcacatttccccgaaaacgtcttcaagctgcctcgcgcgtttcggtgatgacggtgaaaacctctgacacatgcagctcccggagacggtcacagcttgtctgtaagcggatgccgggagcagacaagcccgtcagggcgcgtcagcgggtgttggcgggtgtcggggcgcagccatgacccagtcacgtagcgatagcggagttggcttaactatgcggcatcagagcagattgtactgagagtgcaccatatcgacgctctcccttatgcgactcctgcattaggaagcagcccagtagtaggttgaggccgttgagcaccgccgccgcaaggaatggtgctggcttatcgaaattaatcgactcactatagggagaccc

SEQ ID NO: 23 - DNA, 4337 bp, Artificial Sequence
  plasmids encoding empty vector
gaattcgagctcgccccgttacataacttacggtaaatggcccgcctggctgaccgcccaacgacccccgcccattgacgtcaataatgacgtatgttcccatagtaacgccaatagggactttccattgacgtcaatgggtggagtatttacggtaaactgcccacttggcagtacatcaagtgtatcatatgccaagtacgccccctattgacgtcaatgacggtaaatggcccgcctggcattatgcccagtacatgaccttatgggactttcctacttggcagtacatctacgtattagtcatcgctattaccatggtgatgcggttttggcagtacatcaatgggcgtggatagcggtttgactcacggggatttccaagtctccaccccattgacgtcaatgggagtttgttttggcaccaaaatcaacgggactttccaaaatgtcgtaacaactccgccccattgacgcaaatgggcggtaggcgtgtacggtgggaggtctatataagcagagctcgtttagtgaaccgtcagatcgcctggagacgccatccacgctgttttgacctccatagaagacaccgggaccgatccagcctccgggggatcgatcccccgatcctgagaacttcagggtgagtttggggacccttgattgttctttctttttcgctattgtaaaattcatgttatatggagggggcaaagttttcagggtgttgtttagaatgggaagatgtcccttgtatcaccatggaccctcatgataattttgtttctttcactttctactctgttgacaaccattgtctcctcttattttcttttcattttctgtaactttttcgttaaactttagcttgcatttgtaacgaatttttaaattcacttttgtttatttgtcagattgtaagtactttctctaatcacttttttttcaaggcaatcagggtatattatattgtacttcagcacagttttagagaacaattgttataattaaatgataaggtagaatatttctgcatataaattctggctggcgtggaaatattcttattggtagaaacaactacatcctggtcatcatcctgcctttctctttatggttacaatgatatacactgtttgagatgaggataaaatactctgagtccaaaccgggcccctctgctaaccatgttcatgccttcttctttttcctacagctcctgggcaacgtgctggttattgtgctgtctcatcattttggcaaagaattgtaatacgactcactatagggcgaattcggatccgccacctctagagtcgactgtttaaacctgcaggcatgcaagctgatctttttccctctgccaaaaattatggggacatcatgaagccccttgagcatctgacttctggctaataaaggaaatttattttcattgcaatagtgtgttggaattttttgtgtctctcactcggaaggacatatgggagggcaaatcatttaaaacatcagaatgagtatttggtttagagtttggcaacatatgccatatgctggctgccatgaacaaaggtggctataaagaggtcatcagtatatgaaacagccccctgctgtccattccttattccatagaaaagccttgacttgaggttagattttttttatattttgttttgtgttatttttttctttaacatccctaaaattttccttacatgttttactagccagatttttcctcctctcctgactactcccagtcatagctgtccctcttctcttatgaactcgaggagctttttgcaaaagcctaggcctccaaaaaagcctcctcactacttctggaatagctcagaggccgaggcggcctcggcctctgcataaataaaaaaaattagtcagccatggggcggagaatgggcggaactgggcggagttaggggcgggatgggcggagttaggggcgggactatggttgctgactaattgagactgcattaatgaatcggccaacgcgcggggagaggcggtttgcgtattgggcgctcttccgcttcctcgctcactgactcgctgcgctcggtcgttcggctgcggcgagcggtatcagctcactcaaaggcggtaatacggttatccacagaatcaggggataacgcaggaaagaacatgtgagcaaaaggccagcaaaaggccaggaaccgtaaaaaggccgcgttgctggcgtttttccataggctccgcccccctgacgagcatcacaaaaatcgacgctcaagtcagaggtggcgaaacccgacaggactataaagataccaggcgtttccccctggaagctccctcgtgcgctctcctgttccgaccctgccgcttaccggatacctgtccgcctttctcccttcgggaagcgtggcgctttctcaatgctcacgctgtaggtatctcagttcggtgtaggtcgttcgctccaagctgggctgtgtgcacgaaccccccgttcagcccgaccgctgcgccttatccggtaactatcgtcttgagtccaacccggtaagacacgacttatcgccactggcagcagccactggtaacaggattagcagagcgaggtatgtaggcggtgctacagagttcttgaagtggtggcctaactacggctacactagaaggacagtatttggtatctgcgctctgctgaagccagttaccttcggaaaaagagttggtagctcttgatccggcaaacaaaccaccgctggtagcggtggtttttttgtttgcaagcagcagattacgcgcagaaaaaaaggatctcaagaagatcctttgatcttttctacggggtctgacgctcagtggaacgaaaactcacgttaagggattttggtcatgagattatcaaaaaggatcttcacctagatccttttaaattaaaaatgaagttttaaatcaatctaaagtatatatgagtaaacttggtctgacagttaccaatgcttaatcagtgaggcacctatctcagcgatctgtctatttcgttcatccatagttgcctgactccccgtcgtgtagataactacgatacgggagggcttaccatctggccccagtgctgcaatgataccgcgagacccacgctcaccggctccagatttatcagcaataaaccagccagccggaagggccgagcgcagaagtggtcctgcaactttatccgcctccatccagtctattaattgttgccgggaagctagagtaagtagttcgccagttaatagtttgcgcaacgttgttgccattgctacaggcatcgtggtgtcacgctcgtcgtttggtatggcttcattcagctccggttcccaacgatcaaggcgagttacatgatcccccatgttgtgcaaaaaagcggttagctccttcggtcctccgatcgttgtcagaagtaagttggccgcagtgttatcactcatggttatggcagcactgcataattctcttactgtcatgccatccgtaagatgcttttctgtgactggtgagtactcaaccaagtcattctgagaatagtgtatgcggcgaccgagttgctcttgcccggcgtcaatacgggataataccgcgccacatagcagaactttaaaagtgctcatcattggaaaacgttcttcggggcgaaaactctcaaggatcttaccgctgttgagatccagttcgatgtaacccactcgtgcacccaactgatcttcagcatcttttactttcaccagcgtttctgggtgagcaaaaacaggaaggcaaaatgccgcaaaaaagggaataagggcgacacggaaatgttgaatactcatactcttcctttttcaatattattgaagcatttatcagggttattgtctcatgagcggatacatatttgaatgtatttagaaaaataaacaaataggggttccgcgcacatttccccgaaaacgtcttcaagctgcctcgcgcgtttcggtgatgacggtgaaaacctctgacacatgcagctcccggagacggtcacagcttgtctgtaagcggatgccgggagcagacaagcccgtcagggcgcgtcagcgggtgttggcgggtgtcggggcgcagccatgacccagtcacgtagcgatagcggagttggcttaactatgcggcatcagagcagattgtactgagagtgcaccatatcgacgctctcccttatgcgactcctgcattaggaagcagcccagtagtaggttgaggccgttgagcaccgccgccgcaaggaatggtgctggcttatcgaaattaatcgactcactatagggagaccc

SEQ ID NO: 24 - DNA, 9893 bp, Artificial Sequence
  Vector for ACE2 transduction
acgcgtgtagtcttatgcaatactcttgtagtcttgcaacatggtaacgatgagttagcaacatgccttacaaggagagaaaaagcaccgtgcatgccgattggtggaagtaaggtggtacgatcgtgccttattaggaaggcaacagacgggtctgacatggattggacgaaccactgaattgccgcattgcagagatattgtatttaagtgcctagctcgatacaataaacgggtctctctggttagaccagatctgagcctgggagctctctggctaactagggaacccactgcttaagcctcaataaagcttgccttgagtgcttcaagtagtgtgtgcccgtctgttgtgtgactctggtaactagagatccctcagacccttttagtcagtgtggaaaatctctagcagtggcgcccgaacagggacctgaaagcgaaagggaaaccagagctctctcgacgcaggactcggcttgctgaagcgcgcacggcaagaggcgaggggcggcgactggtgagtacgccaaaaattttgactagcggaggctagaaggagagagatgggtgcgagagcgtcagtattaagcgggggagaattagatcgcgatgggaaaaaattcggttaaggccagggggaaagaaaaaatataaattaaaacatatagtatgggcaagcagggagctagaacgattcgcagttaatcctggcctgttagaaacatcagaaggctgtagacaaatactgggacagctacaaccatcccttcagacaggatcagaagaacttagatcattatataatacagtagcaaccctctattgtgtgcatcaaaggatagagataaaagacaccaaggaagctttagacaagatagaggaagagcaaaacaaaagtaagaccaccgcacagcaagcggccactgatcttcagacctggaggaggagatatgagggacaattggagaagtgaattatataaatataaagtagtaaaaattgaaccattaggagtagcacccaccaaggcaaagagaagagtggtgcagagagaaaaaagagcagtgggaataggagctttgttccttgggttcttgggagcagcaggaagcactatgggcgcagcgtcaatgacgctgacggtacaggccagacaattattgtctggtatagtgcagcagcagaacaatttgctgagggctattgaggcgcaacagcatctgttgcaactcacagtctggggcatcaagcagctccaggcaagaatcctggctgtggaaagatacctaaaggatcaacagctcctggggatttggggttgctctggaaaactcatttgcaccactgctgtgccttggaatgctagttggagtaataaatctctggaacagatttggaatcacacgacctggatggagtgggacagagaaattaacaattacacaagcttaatacactccttaattgaagaatcgcaaaaccagcaagaaaagaatgaacaagaattattggaattagataaatgggcaagtttgtggaattggtttaacataacaaattggctgtggtatataaaattattcataatgatagtaggaggcttggtaggtttaagaatagtttttgctgtactttctatagtgaatagagttaggcagggatattcaccattatcgtttcagacccacctcccaaccccgaggggacccgacaggcccgaaggaatagaagaagaaggtggagagagagacagagacagatccattcgattagtgaacggatctcgacggtatcggttaacttttaaaagaaaaggggggattggggggtacagtgcaggggaaagaatagtagacataatagcaacagacatacaaactaaagaattacaaaaacaaattacaaaattcaaaattttatcgattactagtattatgcccagtacatgaccttatgggactttcctacttggcagtacatctacgtattagtcatcgctattaccatggtgatgcggttttggcagtacatcaatgggcgtggatagcggtttgactcacggggatttccaagtctccaccccattgacgtcaatgggagtttgttttggcaccaaaatcaacgggactttccaaaatgtcgtaacaactccgccccattgacgcaaatgggcggtaggcgtgtacggtgggaggtttatataagcagagctcgtttagtgaaccgtcagatcgcctggagacgccatccacgctgttttgacctccatagaagattctagagctagcgtttaaacttaagcttggtaccgagctcggatccactagtccagtgtggtggaattctgcagatatccagcacagtggcggccgctcgagatgtcaagctcttcctggctccttctcagccttgttgctgtaactgctgctcagtccaccattgaggaacaggccaagacatttttggacaagtttaaccacgaagccgaagacctgttctatcaaagttcacttgcttcttggaattataacaccaatattactgaagagaatgtccaaaacatgaataatgctggggacaaatggtctgcctttttaaaggaacagtccacacttgcccaaatgtatccactacaagaaattcagaatctcacagtcaagcttcagctgcaggctcttcagcaaaatgggtcttcagtgctctcagaagacaagagcaaacggttgaacacaattctaaatacaatgagcaccatctacagtactggaaaagtttgtaacccagataatccacaagaatgcttattacttgaaccaggtttgaatgaaataatggcaaacagtttagactacaatgagaggctctgggcttgggaaagctggagatctgaggtcggcaagcagctgaggccattatatgaagagtatgtggtcttgaaaaatgagatggcaagagcaaatcattatgaggactatggggattattggagaggagactatgaagtaaatggggtagatggctatgactacagccgcggccagttgattgaagatgtggaacatacctttgaagagattaaaccattatatgaacatcttcatgcctatgtgagggcaaagttgatgaatgcctatccttcctatatcagtccaattggatgcctccctgctcatttgcttggtgatatgtggggtagattttggacaaatctgtactctttgacagttccctttggacagaaaccaaacatagatgttactgatgcaatggtggaccaggcctgggatgcacagagaatattcaaggaggccgagaagttctttgtatctgttggtcttcctaatatgactcaaggattctgggaaaattccatgctaacggacccaggaaatgttcagaaagcagtctgccatcccacagcttgggacctggggaagggcgacttcaggatccttatgtgcacaaaggtgacaatggacgacttcctgacagctcatcatgagatggggcatatccagtatgatatggcatatgctgcacaaccttttctgctaagaaatggagctaatgaaggattccatgaagctgttggggaaatcatgtcactttctgcagccacacctaagcatttaaaatccattggtcttctgtcacccgattttcaagaagacaatgaaacagaaataaacttcctgctcaaacaagcactcacgattgttgggactctgccatttacttacatgttagagaagtggaggtggatggtctttaaaggggaaattcccaaagaccagtggatgaaaaagtggtgggagatgaagcgagagatagttggggtggtggaacctgtgccccatgatgaaacatactgtgaccccgcatctctgttccatgtttctaatgattactcattcattcgatattacacaaggaccctttaccaattccagtttcaagaagcactttgtcaagcagctaaacatgaaggccctctgcacaaatgtgacatctcaaactctacagaagctggacagaaactgttcaatatgctgaggcttggaaaatcagaaccctggaccctagcattggaaaatgttgtaggagcaaagaacatgaatgtaaggccactgctcaactactttgagcccttatttacctggctgaaagaccagaacaagaattcttttgtgggatggagtaccgactggagtccatatgcagaccaaagcatcaaagtgaggataagcctaaaatcagctcttggagataaagcatatgaatggaacgacaatgaaatgtacctgttccgatcatctgttgcatatgctatgaggcagtactttttaaaagtaaaaaatcagatgattctttttggggaggaggatgtgcgagtggctaatttgaaaccaagaatctcctttaatttctttgtcactgcacctaaaaatgtgtctgatatcattcctagaactgaagttgaaaaggccatcaggatgtcccggagccgtatcaatgatgctttccgtctgaatgacaacagcctagagtttctggggatacagccaacacttggacctcctaaccagccccctgtttccatatggctgattgtttttggagttgtgatgggagtgatagtggttggcattgtcatcctgatcttcactgggatcagagatcggaagaagaaaaataaagcaagaagtggagaaaatccttatgcctccatcgatattagcaaaggagaaaataatccaggattccaaaacactgatgatgttcagacctccttttagcccaaatcggatccgcggccgcaaggatctgcgatcgctccggtgcccgtcagtgggcagagcgcacatcgcccacagtccccgagaagttggggggaggggtcggcaattgaacgggtgcctagagaaggtggcgcggggtaaactgggaaagtgatgtcgtgtactggctccgcctttttcccgagggtgggggagaaccgtatataagtgcagtagtcgccgtgaacgttctttttcgcaacgggtttgccgccagaacacagctgaagcttcgaggggctcgcatctctccttcacgcgcccgccgccctacctgaggccgccatccacgccggttgagtcgcgttctgccgcctcccgcctgtggtgcctcctgaactgcgtccgccgtctaggtaagtttaaagctcaggtcgagaccgggcctttgtccggcgctcccttggagcctacctagactcagccggctctccacgctttgcctgaccctgcttgctcaactctacgtctttgtttcgttttctgttctgcgccgttacagatccaagctgtgaccggcgcctacgatatgaccgagtacaagcccacggtgcgcctcgccacccgcgacgacgtccccagggccgtacgcaccctcgccgccgcgttcgccgactaccccgccacgcgccacaccgtcgatccggaccgccacatcgagcgggtcaccgagctgcaagaactcttcctcacgcgcgtcgggctcgacatcggcaaggtgtgggtcgcggacgacggcgccgcggtggcggtctggaccacgccggagagcgtcgaagcgggggcggtgttcgccgagatcggcccgcgcatggccgagttgagcggttcccggctggccgcgcagcaacagatggaaggcctcctggcgccgcaccggcccaaggagcccgcgtggttcctggccaccgtcggcgtctcgcccgaccaccagggcaagggtctgggcagcgccgtcgtgctccccggagtggaggcggccgagcgcgccggggtgcccgccttcctggagacctccgcgccccgcaacctccccttctacgagcggctcggcttcaccgtcaccgccgacgtcgaggtgcccgaaggaccgcgcacctggtgcatgacccgcaagcccggtgcctgacaatcaacctctggattacaaaatttgtgaaagattgactggtattcttaactatgttgctccttttacgctatgtggatacgctgctttaatgcctttgtatcatgctattgcttcccgtatggctttcattttctcctccttgtataaatcctggttgctgtctctttatgaggagttgtggcccgttgtcaggcaacgtggcgtggtgtgcactgtgtttgctgacgcaacccccactggttggggcattgccaccacctgtcagctcctttccgggactttcgctttccccctccctattgccacggcggaactcatcgccgcctgccttgcccgctgctggacaggggctcggctgttgggcactgacaattccgtggtgttgtcggggaaatcatcgtcctttccttggctgctcgcctgtgttgccacctggattctgcgcgggacgtccttctgctacgtcccttcggccctcaatccagcggaccttccttcccgcggcctgctgccggctctgcggcctcttccgcgtcttcgccttcgccctcagacgagtcggatctccctttgggccgcctccccgcctggtacctttaagaccaatgacttacaaggcagctgtagatcttagccactttttaaaagaaaaggggggactggaagggctaattcactcccaacgaagataagatctgctttttgcttgtactgggtctctctggttagaccagatctgagcctgggagctctctggctaactagggaacccactgcttaagcctcaataaagcttgccttgagtgcttcaagtagtgtgtgcccgtctgttgtgtgactctggtaactagagatccctcagacccttttagtcagtgtggaaaatctctagcagtagtagttcatgtcatcttattattcagtatttataacttgcaaagaaatgaatatcagagagtgagaggaacttgtttattgcagcttataatggttacaaataaagcaatagcatcacaaatttcacaaataaagcatttttttcactgcattctagttgtggtttgtccaaactcatcaatgtatcttatcatgtctggctctagctatcccgcccctaactccgcccatcccgcccctaactccgcccagttccgcccattctccgccccatggctgactaattttttttatttatgcagaggccgaggccgcctcggcctctgagctattccagaagtagtgaggaggcttttttggaggcctagacttttgcagagaccaaattcgtaatcatgtcatagctgtttcctgtgtgaaattgttatccgctcacaattccacacaacatacgagccggaagcataaagtgtaaagcctggggtgcctaatgagtgagctaactcacattaattgcgttgcgctcactgcccgctttccagtcgggaaacctgtcgtgccagctgcattaatgaatcggccaacgcgcggggagaggcggtttgcgtattgggcgctcttccgcttcctcgctcactgactcgctgcgctcggtcgttcggctgcggcgagcggtatcagctcactcaaaggcggtaatacggttatccacagaatcaggggataacgcaggaaagaacatgtgagcaaaaggccagcaaaaggccaggaaccgtaaaaaggccgcgttgctggcgtttttccataggctccgcccccctgacgagcatcacaaaaatcgacgctcaagtcagaggtggcgaaacccgacaggactataaagataccaggcgtttccccctggaagctccctcgtgcgctctcctgttccgaccctgccgcttaccggatacctgtccgcctttctcccttcgggaagcgtggcgctttctcatagctcacgctgtaggtatctcagttcggtgtaggtcgttcgctccaagctgggctgtgtgcacgaaccccccgttcagcccgaccgctgcgccttatccggtaactatcgtcttgagtccaacccggtaagacacgacttatcgccactggcagcagccactggtaacaggattagcagagcgaggtatgtaggcggtgctacagagttcttgaagtggtggcctaactacggctacactagaaggacagtatttggtatctgcgctctgctgaagccagttaccttcggaaaaagagttggtagctcttgatccggcaaacaaaccaccgctggtagcggtggtttttttgtttgcaagcagcagattacgcgcagaaaaaaaggatctcaagaagatcctttgatcttttctacggggtctgacgctcagtggaacgaaaactcacgttaagggattttggtcatgagattatcaaaaaggatcttcacctagatccttttaaattaaaaatgaagttttaaatcaatctaaagtatatatgagtaaacttggtctgacagttaccaatgcttaatcagtgaggcacctatctcagcgatctgtctatttcgttcatccatagttgcctgactccccgtcgtgtagataactacgatacgggagggcttaccatctggccccagtgctgcaatgataccgcgagacccacgctcaccggctccagatttatcagcaataaaccagccagccggaagggccgagcgcagaagtggtcctgcaactttatccgcctccatccagtctattaattgttgccgggaagctagagtaagtagttcgccagttaatagtttgcgcaacgttgttgccattgctacaggcatcgtggtgtcacgctcgtcgtttggtatggcttcattcagctccggttcccaacgatcaaggcgagttacatgatcccccatgttgtgcaaaaaagcggttagctccttcggtcctccgatcgttgtcagaagtaagttggccgcagtgttatcactcatggttatggcagcactgcataattctcttactgtcatgccatccgtaagatgcttttctgtgactggtgagtactcaaccaagtcattctgagaatagtgtatgcggcgaccgagttgctcttgcccggcgtcaatacgggataataccgcgccacatagcagaactttaaaagtgctcatcattggaaaacgttcttcggggcgaaaactctcaaggatcttaccgctgttgagatccagttcgatgtaacccactcgtgcacccaactgatcttcagcatcttttactttcaccagcgtttctgggtgagcaaaaacaggaaggcaaaatgccgcaaaaaagggaataagggcgacacggaaatgttgaatactcatactcttcctttttcaatattattgaagcatttatcagggttattgtctcatgagcggatacatatttgaatgtatttagaaaaataaacaaataggggttccgcgcacatttccccgaaaagtgccacctgacgtctaagaaaccattattatcatgacattaacctataaaaataggcgtatcacgaggccctttcgtctcgcgcgtttcggtgatgacggtgaaaacctctgacacatgcagctcccggagacggtcacagcttgtctgtaagcggatgccgggagcagacaagcccgtcagggcgcgtcagcgggtgttggcgggtgtcggggctggcttaactatgcggcatcagagcagattgtactgagagtgcaccatatgcggtgtgaaataccgcacagatgcgtaaggagaaaataccgcatcaggcgccattcgccattcaggctgcgcaactgttgggaagggcgatcggtgcgggcctcttcgctattacgccagctggcgaaagggggatgtgctgcaaggcgattaagttgggtaacgccagggttttcccagtcacgacgttgtaaaacgacggccagtgccaagctg

SEQ ID NO: 25 - DNA, 8668 bp, Artificial Sequence
  Vector for TMPRSS2 transduction
acgcgtgtagtcttatgcaatactcttgtagtcttgcaacatggtaacgatgagttagcaacatgccttacaaggagagaaaaagcaccgtgcatgccgattggtggaagtaaggtggtacgatcgtgccttattaggaaggcaacagacgggtctgacatggattggacgaaccactgaattgccgcattgcagagatattgtatttaagtgcctagctcgatacaataaacgggtctctctggttagaccagatctgagcctgggagctctctggctaactagggaacccactgcttaagcctcaataaagcttgccttgagtgcttcaagtagtgtgtgcccgtctgttgtgtgactctggtaactagagatccctcagacccttttagtcagtgtggaaaatctctagcagtggcgcccgaacagggacctgaaagcgaaagggaaaccagagctctctcgacgcaggactcggcttgctgaagcgcgcacggcaagaggcgaggggcggcgactggtgagtacgccaaaaattttgactagcggaggctagaaggagagagatgggtgcgagagcgtcagtattaagcgggggagaattagatcgcgatgggaaaaaattcggttaaggccagggggaaagaaaaaatataaattaaaacatatagtatgggcaagcagggagctagaacgattcgcagttaatcctggcctgttagaaacatcagaaggctgtagacaaatactgggacagctacaaccatcccttcagacaggatcagaagaacttagatcattatataatacagtagcaaccctctattgtgtgcatcaaaggatagagataaaagacaccaaggaagctttagacaagatagaggaagagcaaaacaaaagtaagaccaccgcacagcaagcggccactgatcttcagacctggaggaggagatatgagggacaattggagaagtgaattatataaatataaagtagtaaaaattgaaccattaggagtagcacccaccaaggcaaagagaagagtggtgcagagagaaaaaagagcagtgggaataggagctttgttccttgggttcttgggagcagcaggaagcactatgggcgcagcgtcaatgacgctgacggtacaggccagacaattattgtctggtatagtgcagcagcagaacaatttgctgagggctattgaggcgcaacagcatctgttgcaactcacagtctggggcatcaagcagctccaggcaagaatcctggctgtggaaagatacctaaaggatcaacagctcctggggatttggggttgctctggaaaactcatttgcaccactgctgtgccttggaatgctagttggagtaataaatctctggaacagatttggaatcacacgacctggatggagtgggacagagaaattaacaattacacaagcttaatacactccttaattgaagaatcgcaaaaccagcaagaaaagaatgaacaagaattattggaattagataaatgggcaagtttgtggaattggtttaacataacaaattggctgtggtatataaaattattcataatgatagtaggaggcttggtaggtttaagaatagtttttgctgtactttctatagtgaatagagttaggcagggatattcaccattatcgtttcagacccacctcccaaccccgaggggacccgacaggcccgaaggaatagaagaagaaggtggagagagagacagagacagatccattcgattagtgaacggatctcgacggtatcggttaacttttaaaagaaaaggggggattggggggtacagtgcaggggaaagaatagtagacataatagcaacagacatacaaactaaagaattacaaaaacaaattacaaaattcaaaattttatcgattactagtattatgcccagtacatgaccttatgggactttcctacttggcagtacatctacgtattagtcatcgctattaccatggtgatgcggttttggcagtacatcaatgggcgtggatagcggtttgactcacggggatttccaagtctccaccccattgacgtcaatgggagtttgttttggcaccaaaatcaacgggactttccaaaatgtcgtaacaactccgccccattgacgcaaatgggcggtaggcgtgtacggtgggaggtttatataagcagagctcgtttagtgaaccgtcagatcgcctggagacgccatccacgctgttttgacctccatagaagattctagagctagcgtttaaacttaaggccaccatggctttgaactcagggtcaccaccagctattggaccttactatgaaaaccatggataccaaccggaaaacccctatcccgcacagcccactgtggtccccactgtctacgaggtgcatccggctcagtactacccgtcccccgtgccccagtacgccccgagggtcctgacgcaggcttccaaccccgtcgtctgcacgcagcccaaatccccatccgggacagtgtgcacctcaaagactaagaaagcactgtgcatcaccttgaccctggggaccttcctcgtgggagctgcgctggccgctggcctactctggaagttcatgggcagcaagtgctccaactctgggatagagtgcgactcctcaggtacctgcatcaacccctctaactggtgtgatggcgtgtcacactgccccggcggggaggacgagaatcggtgtgttcgcctctacggaccaaacttcatccttcaggtgtactcatctcagaggaagtcctggcaccctgtgtgccaagacgactggaacgagaactacgggcgggcggcctgcagggacatgggctataagaataatttttactctagccaaggaatagtggatgacagcggatccaccagctttatgaaactgaacacaagtgccggcaatgtcgatatctataaaaaactgtaccacagtgatgcctgttcttcaaaagcagtggtttctttacgctgtatagcctgcggggtcaacttgaactcaagccgccagagcaggattgtgggcggcgagagcgcgctcccgggggcctggccctggcaggtcagcctgcacgtccagaacgtccacgtgtgcggaggctccatcatcacccccgagtggatcgtgacagccgcccactgcgtggaaaaacctcttaacaatccatggcattggacggcatttgcggggattttgagacaatctttcatgttctatggagccggataccaagtagaaaaagtgatttctcatccaaattatgactccaagaccaagaacaatgacattgcgctgatgaagctgcagaagcctctgactttcaacgacctagtgaaaccagtgtgtctgcccaacccaggcatgatgctgcagccagaacagctctgctggatttccgggtggggggccaccgaggagaaagggaagacctcagaagtgctgaacgctgccaaggtgcttctcattgagacacagagatgcaacagcagatatgtctatgacaacctgatcacaccagccatgatctgtgccggcttcctgcaggggaacgtcgattcttgccagggtgacagtggagggcctctggtcacttcgaagaacaatatctggtggctgataggggatacaagctggggttctggctgtgccaaagcttacagaccaggagtgtacgggaatgtgatggtattcacggactggatttatcgacaaatgagggcagacggctaagcggccgcaaggatctgcgatcgctccggtgcccgtcagtgggcagagcgcacatcgcccacagtccccgagaagttggggggaggggtcggcaattgaacgggtgcctagagaaggtggcgcggggtaaactgggaaagtgatgtcgtgtactggctccgcctttttcccgagggtgggggagaaccgtatataagtgcagtagtcgccgtgaacgttctttttcgcaacgggtttgccgccagaacacagctgaagcttcgaggggctcgcatctctccttcacgcgcccgccgccctacctgaggccgccatccacgccggttgagtcgcgttctgccgcctcccgcctgtggtgcctcctgaactgcgtccgccgtctaggtaagtttaaagctcaggtcgagaccgggcctttgtccggcgctcccttggagcctacctagactcagccggctctccacgctttgcctgaccctgcttgctcaactctacgtctttgtttcgttttctgttctgcgccgttacagatccaagctgtgaccggcgcctacgatatggccaagcctttgtctcaagaagaatccaccctcattgaaagagcaacggctacaatcaacagcatccccatctctgaagactacagcgtcgccagcgcagctctctctagcgacggccgcatcttcactggtgtcaatgtatatcattttactgggggaccttgtgcagaactcgtggtgctgggcactgctgctgctgcggcagctggcaacctgacttgtatcgtcgcgatcggaaatgagaacaggggcatcttgagcccctgcggacggtgccgacaggtgcttctcgatctgcatcctgggatcaaagccatagtgaaggacagtgatggacagccgacggcagttgggattcgtgaattgctgccctctggttatgtgtgggagggctaacaatcaacctctggattacaaaatttgtgaaagattgactggtattcttaactatgttgctccttttacgctatgtggatacgctgctttaatgcctttgtatcatgctattgcttcccgtatggctttcattttctcctccttgtataaatcctggttgctgtctctttatgaggagttgtggcccgttgtcaggcaacgtggcgtggtgtgcactgtgtttgctgacgcaacccccactggttggggcattgccaccacctgtcagctcctttccgggactttcgctttccccctccctattgccacggcggaactcatcgccgcctgccttgcccgctgctggacaggggctcggctgttgggcactgacaattccgtggtgttgtcggggaaatcatcgtcctttccttggctgctcgcctgtgttgccacctggattctgcgcgggacgtccttctgctacgtcccttcggccctcaatccagcggaccttccttcccgcggcctgctgccggctctgcggcctcttccgcgtcttcgccttcgccctcagacgagtcggatctccctttgggccgcctccccgcctggtacctttaagaccaatgacttacaaggcagctgtagatcttagccactttttaaaagaaaaggggggactggaagggctaattcactcccaacgaagataagatctgctttttgcttgtactgggtctctctggttagaccagatctgagcctgggagctctctggctaactagggaacccactgcttaagcctcaataaagcttgccttgagtgcttcaagtagtgtgtgcccgtctgttgtgtgactctggtaactagagatccctcagacccttttagtcagtgtggaaaatctctagcagtagtagttcatgtcatcttattattcagtatttataacttgcaaagaaatgaatatcagagagtgagaggaacttgtttattgcagcttataatggttacaaataaagcaatagcatcacaaatttcacaaataaagcatttttttcactgcattctagttgtggtttgtccaaactcatcaatgtatcttatcatgtctggctctagctatcccgcccctaactccgcccatcccgcccctaactccgcccagttccgcccattctccgccccatggctgactaattttttttatttatgcagaggccgaggccgcctcggcctctgagctattccagaagtagtgaggaggcttttttggaggcctagacttttgcagagaccaaattcgtaatcatgtcatagctgtttcctgtgtgaaattgttatccgctcacaattccacacaacatacgagccggaagcataaagtgtaaagcctggggtgcctaatgagtgagctaactcacattaattgcgttgcgctcactgcccgctttccagtcgggaaacctgtcgtgccagctgcattaatgaatcggccaacgcgcggggagaggcggtttgcgtattgggcgctcttccgcttcctcgctcactgactcgctgcgctcggtcgttcggctgcggcgagcggtatcagctcactcaaaggcggtaatacggttatccacagaatcaggggataacgcaggaaagaacatgtgagcaaaaggccagcaaaaggccaggaaccgtaaaaaggccgcgttgctggcgtttttccataggctccgcccccctgacgagcatcacaaaaatcgacgctcaagtcagaggtggcgaaacccgacaggactataaagataccaggcgtttccccctggaagctccctcgtgcgctctcctgttccgaccctgccgcttaccggatacctgtccgcctttctcccttcgggaagcgtggcgctttctcatagctcacgctgtaggtatctcagttcggtgtaggtcgttcgctccaagctgggctgtgtgcacgaaccccccgttcagcccgaccgctgcgccttatccggtaactatcgtcttgagtccaacccggtaagacacgacttatcgccactggcagcagccactggtaacaggattagcagagcgaggtatgtaggcggtgctacagagttcttgaagtggtggcctaactacggctacactagaaggacagtatttggtatctgcgctctgctgaagccagttaccttcggaaaaagagttggtagctcttgatccggcaaacaaaccaccgctggtagcggtggtttttttgtttgcaagcagcagattacgcgcagaaaaaaaggatctcaagaagatcctttgatcttttctacggggtctgacgctcagtggaacgaaaactcacgttaagggattttggtcatgagattatcaaaaaggatcttcacctagatccttttaaattaaaaatgaagttttaaatcaatctaaagtatatatgagtaaacttggtctgacagttaccaatgcttaatcagtgaggcacctatctcagcgatctgtctatttcgttcatccatagttgcctgactccccgtcgtgtagataactacgatacgggagggcttaccatctggccccagtgctgcaatgataccgcgagacccacgctcaccggctccagatttatcagcaataaaccagccagccggaagggccgagcgcagaagtggtcctgcaactttatccgcctccatccagtctattaattgttgccgggaagctagagtaagtagttcgccagttaatagtttgcgcaacgttgttgccattgctacaggcatcgtggtgtcacgctcgtcgtttggtatggcttcattcagctccggttcccaacgatcaaggcgagttacatgatcccccatgttgtgcaaaaaagcggttagctccttcggtcctccgatcgttgtcagaagtaagttggccgcagtgttatcactcatggttatggcagcactgcataattctcttactgtcatgccatccgtaagatgcttttctgtgactggtgagtactcaaccaagtcattctgagaatagtgtatgcggcgaccgagttgctcttgcccggcgtcaatacgggataataccgcgccacatagcagaactttaaaagtgctcatcattggaaaacgttcttcggggcgaaaactctcaaggatcttaccgctgttgagatccagttcgatgtaacccactcgtgcacccaactgatcttcagcatcttttactttcaccagcgtttctgggtgagcaaaaacaggaaggcaaaatgccgcaaaaaagggaataagggcgacacggaaatgttgaatactcatactcttcctttttcaatattattgaagcatttatcagggttattgtctcatgagcggatacatatttgaatgtatttagaaaaataaacaaataggggttccgcgcacatttccccgaaaagtgccacctgacgtctaagaaaccattattatcatgacattaacctataaaaataggcgtatcacgaggccctttcgtctcgcgcgtttcggtgatgacggtgaaaacctctgacacatgcagctcccggagacggtcacagcttgtctgtaagcggatgccgggagcagacaagcccgtcagggcgcgtcagcgggtgttggcgggtgtcggggctggcttaactatgcggcatcagagcagattgtactgagagtgcaccatatgcggtgtgaaataccgcacagatgcgtaaggagaaaataccgcatcaggcgccattcgccattcaggctgcgcaactgttgggaagggcgatcggtgcgggcctcttcgctattacgccagctggcgaaagggggatgtgctgcaaggcgattaagttgggtaacgccagggttttcccagtcacgacgttgtaaaacgacggccagtgccaagctg

SEQ ID NO: 26 - DNA, 23 bp, Artificial Sequence
  ACE2 forward primer
cattggagcaagtgttggatctt

SEQ ID NO: 27 - DNA, 22 bp, Artificial Sequence
  ACE2 reverse primer
gagctaatgcatgccattctca

SEQ ID NO: 28 - DNA, 22 bp, Artificial Sequence
  TMPRSS2 forward primer
cacggactggatttatcgacaa

SEQ ID NO: 29 - DNA, 21 bp, Artificial Sequence
  TMPRSS2 reverse primer
cgtcaaggacgaagaccatgt

SEQ ID NO: 30 - DNA, 22 bp, Artificial Sequence
  GAPDH forward primer
gcacaagaggaagagagagacc

SEQ ID NO: 31 - DNA, 20 bp, Artificial Sequence
  GAPDH reverse primer
aggggagattcagtgtggtg

SEQ ID NO: 32 - DNA, 20 bp, Artificial Sequence
  Furin Forward
ggaacatgacagctgcaact

SEQ ID NO: 33 - DNA, 20 bp, Artificial Sequence
  Furin Reverse
tcgtcacgatctgcttctca

SEQ ID NO: 34 - DNA, 20 bp, Artificial Sequence
  Cathepsin L Forward
tagaggcacagtggaccaag

SEQ ID NO: 35 - DNA, 20 bp, Artificial Sequence
  Cathepsin L Reverse
atggccattgtgaagctgtg

SEQ ID NO: 36 - DNA, 20 bp, Artificial Sequence
  Cathepsin B Forward
tctctgaccggatctgcatc

SEQ ID NO: 37 - DNA, 20 bp, Artificial Sequence
  Cathepsin B Reverse
tcacagggagggatggagta

SEQ ID NO: 38 - DNA, 20 bp, Artificial Sequence
  PC1 Forward
gcgtgcctgagaagaaagag

SEQ ID NO: 39 - DNA, 20 bp, Artificial Sequence
  PC1 Reverse
atcccgttctctttcagcca

SEQ ID NO: 40 - DNA, 20 bp, Artificial Sequence
  Trypsin Forward
aagtgtgaagcctcctaccc

SEQ ID NO: 41 - DNA, 20 bp, Artificial Sequence
  Trypsin Reverse
ggtgtagactccaggcttgt

SEQ ID NO: 42 - DNA, 20 bp, Artificial Sequence
  Matriptase Forward
cccaacaaccagcatgtgaa

SEQ ID NO: 43 - DNA, 20 bp, Artificial Sequence
  Matriptase Reverse
actggagtcgtaggagaggt

SEQ ID NO: 44 - DNA, 20 bp, Artificial Sequence
  Matriptase Forward
agaacgtcctgctcatcaca

SEQ ID NO: 45 - DNA, 20 bp, Artificial Sequence
  Matriptase Reverse
tgtgcagtcaatgttgggtg

SEQ ID NO: 46 - DNA, 6623 bp, Artificial Sequence
  HEK293 AAT Vector
gacggatcgggagatctcccgatcccctatggtgcactctcagtacaatctgctctgatgccgcatagttaagccagtatctgctccctgcttgtgtgttggaggtcgctgagtagtgcgcgagcaaaatttaagctacaacaaggcaaggcttgaccgacaattgcatgaagaatctgcttagggttaggcgttttgcgctgcttcgcgatgtacgggccagatatacgcgttgacattgattattgactagttattaatagtaatcaattacggggtcattagttcatagcccatatatggagttccgcgttacataacttacggtaaatggcccgcctggctgaccgcccaacgacccccgcccattgacgtcaataatgacgtatgttcccatagtaacgccaatagggactttccattgacgtcaatgggtggagtatttacggtaaactgcccacttggcagtacatcaagtgtatcatatgccaagtacgccccctattgacgtcaatgacggtaaatggcccgcctggcattatgcccagtacatgaccttatgggactttcctacttggcagtacatctacgtattagtcatcgctattaccatggtgatgcggttttggcagtacatcaatgggcgtggatagcggtttgactcacggggatttccaagtctccaccccattgacgtcaatgggagtttgttttggcaccaaaatcaacgggactttccaaaatgtcgtaacaactccgccccattgacgcaaatgggcggtaggcgtgtacggtgggaggtctatataagcagagctctctggctaactagagaacccactgcttactggcttatcgaaattaatacgactcactatagggagacccaagctggctagcgtttaaacttaagcttgccaccatgccgtcttctgtctcgtggggcatcctcctgctggcaggcctgtgctgcctggtccctgtctccctggctgaggatccccagggagatgctgcccagaagacagatacatcccaccatgatcaggatcacccaaccttcaacaagatcacccccaacctggctgagttcgccttcagcctataccgccagctggcacaccagtccaacagcaccaatatcttcttctccccagtgagcatcgctacagcctttgcaatgctctccctggggaccaaggctgacactcacgatgaaatcctggagggcctgaatttcaacctcacggagattccggaggctcagatccatgaaggcttccaggaactcctccgtaccctcaaccagccagacagccagctccagctgaccaccggcaatggcctgttcctcagcgagggcctgaagctagtggataagtttttggaggatgttaaaaagttgtaccactcagaagccttcactgtcaacttcggggacaccgaagaggccaagaaacagatcaacgattacgtggagaagggtactcaagggaaaattgtggatttggtcaaggagcttgacagagacacagtttttgctctggtgaattacatcttctttaaaggcaaatgggagagaccctttgaagtcaaggacaccgaggaagaggacttccacgtggaccaggtgaccaccgtgaaggtgcctatgatgaagcgtttaggcatgtttaacatccagcactgtaagaagctgtccagctgggtgctgctgatgaaatacctgggcaatgccaccgccatcttcttcctgcctgatgaggggaaactacagcacctggaaaatgaactcacccacgatatcatcaccaagttcctggaaaatgaagacagaaggtctgccagcttacatttacccaaactgtccattactggaacctatgatctgaagagcgtcctgggtcaactgggcatcactaaggtcttcagcaatggggctgacctctccggggtcacagaggaggcacccctgaagctctccaaggccgtgcataaggctgtgctgaccatcgacgagaaagggactgaagctgctggggccatgtttttagaggccatacccatgtctatcccccccgaggtcaagttcaacaaaccctttgtcttcttaatgattgaacaaaataccaagtctcccctcttcatgggaaaagtggtgaatcccacccaaaaataactcgagtctagagggcccgtttaaacccgctgatcagcctcgactgtgccttctagttgccagccatctgttgtttgcccctcccccgtgccttccttgaccctggaaggtgccactcccactgtcctttcctaataaaatgaggaaattgcatcgcattgtctgagtaggtgtcattctattctggggggtggggtggggcaggacagcaagggggaggattgggaagacaatagcaggcatgctggggatgcggtgggctctatggcttctgaggcggaaagaaccagctggggctctagggggtatccccacgcgccctgtagcggcgcattaagcgcggcgggtgtggtggttacgcgcagcgtgaccgctacacttgccagcgccctagcgcccgctcctttcgctttcttcccttcctttctcgccacgttcgccggctttccccgtcaagctctaaatcgggggctccctttagggttccgatttagtgctttacggcacctcgaccccaaaaaacttgattagggtgatggttcacgtagtgggccatcgccctgatagacggtttttcgccctttgacgttggagtccacgttctttaatagtggactcttgttccaaactggaacaacactcaaccctatctcggtctattcttttgatttataagggattttgccgatttcggcctattggttaaaaaatgagctgatttaacaaaaatttaacgcgaattaattctgtggaatgtgtgtcagttagggtgtggaaagtccccaggctccccagcaggcagaagtatgcaaagcatgcatctcaattagtcagcaaccaggtgtggaaagtccccaggctccccagcaggcagaagtatgcaaagcatgcatctcaattagtcagcaaccatagtcccgcccctaactccgcccatcccgcccctaactccgcccagttccgcccattctccgccccatggctgactaattttttttatttatgcagaggccgaggccgcctctgcctctgagctattccagaagtagtgaggaggcttttttggaggcctaggcttttgcaaaaagctcccgggagcttgtatatccattttcggatctgatcaagagacaggatgaggatcgtttcgcatgattgaacaagatggattgcacgcaggttctccggccgcttgggtggagaggctattcggctatgactgggcacaacagacaatcggctgctctgatgccgccgtgttccggctgtcagcgcaggggcgcccggttctttttgtcaagaccgacctgtccggtgccctgaatgaactgcaggacgaggcagcgcggctatcgtggctggccacgacgggcgttccttgcgcagctgtgctcgacgttgtcactgaagcgggaagggactggctgctattgggcgaagtgccggggcaggatctcctgtcatctcaccttgctcctgccgagaaagtatccatcatggctgatgcaatgcggcggctgcatacgcttgatccggctacctgcccattcgaccaccaagcgaaacatcgcatcgagcgagcacgtactcggatggaagccggtcttgtcgatcaggatgatctggacgaagagcatcaggggctcgcgccagccgaactgttcgccaggctcaaggcgcgcatgcccgacggcgaggatctcgtcgtgacccatggcgatgcctgcttgccgaatatcatggtggaaaatggccgcttttctggattcatcgactgtggccggctgggtgtggcggaccgctatcaggacatagcgttggctacccgtgatattgctgaagagcttggcggcgaatgggctgaccgcttcctcgtgctttacggtatcgccgctcccgattcgcagcgcatcgccttctatcgccttcttgacgagttcttctgagcgggactctggggttcgaaatgaccgaccaagcgacgcccaacctgccatcacgagatttcgattccaccgccgccttctatgaaaggttgggcttcggaatcgttttccgggacgccggctggatgatcctccagcgcggggatctcatgctggagttcttcgcccaccccaacttgtttattgcagcttataatggttacaaataaagcaatagcatcacaaatttcacaaataaagcatttttttcactgcattctagttgtggtttgtccaaactcatcaatgtatcttatcatgtctgtataccgtcgacctctagctagagcttggcgtaatcatggtcatagctgtttcctgtgtgaaattgttatccgctcacaattccacacaacatacgagccggaagcataaagtgtaaagcctggggtgcctaatgagtgagctaactcacattaattgcgttgcgctcactgcccgctttccagtcgggaaacctgtcgtgccagctgcattaatgaatcggccaacgcgcggggagaggcggtttgcgtattgggcgctcttccgcttcctcgctcactgactcgctgcgctcggtcgttcggctgcggcgagcggtatcagctcactcaaaggcggtaatacggttatccacagaatcaggggataacgcaggaaagaacatgtgagcaaaaggccagcaaaaggccaggaaccgtaaaaaggccgcgttgctggcgtttttccataggctccgcccccctgacgagcatcacaaaaatcgacgctcaagtcagaggtggcgaaacccgacaggactataaagataccaggcgtttccccctggaagctccctcgtgcgctctcctgttccgaccctgccgcttaccggatacctgtccgcctttctcccttcgggaagcgtggcgctttctcatagctcacgctgtaggtatctcagttcggtgtaggtcgttcgctccaagctgggctgtgtgcacgaaccccccgttcagcccgaccgctgcgccttatccggtaactatcgtcttgagtccaacccggtaagacacgacttatcgccactggcagcagccactggtaacaggattagcagagcgaggtatgtaggcggtgctacagagttcttgaagtggtggcctaactacggctacactagaagaacagtatttggtatctgcgctctgctgaagccagttaccttcggaaaaagagttggtagctcttgatccggcaaacaaaccaccgctggtagcggtttttttgtttgcaagcagcagattacgcgcagaaaaaaaggatctcaagaagatcctttgatcttttctacggggtctgacgctcagtggaacgaaaactcacgttaagggattttggtcatgagattatcaaaaaggatcttcacctagatccttttaaattaaaaatgaagttttaaatcaatctaaagtatatatgagtaaacttggtctgacagttaccaatgcttaatcagtgaggcacctatctcagcgatctgtctatttcgttcatccatagttgcctgactccccgtcgtgtagataactacgatacgggagggcttaccatctggccccagtgctgcaatgataccgcgagacccacgctcaccggctccagatttatcagcaataaaccagccagccggaagggccgagcgcagaagtggtcctgcaactttatccgcctccatccagtctattaattgttgccgggaagctagagtaagtagttcgccagttaatagtttgcgcaacgttgttgccattgctacaggcatcgtggtgtcacgctcgtcgtttggtatggcttcattcagctccggttcccaacgatcaaggcgagttacatgatcccccatgttgtgcaaaaaagcggttagctccttcggtcctccgatcgttgtcagaagtaagttggccgcagtgttatcactcatggttatggcagcactgcataattctcttactgtcatgccatccgtaagatgcttttctgtgactggtgagtactcaaccaagtcattctgagaatagtgtatgcggcgaccgagttgctcttgcccggcgtcaatacgggataataccgcgccacatagcagaactttaaaagtgctcatcattggaaaacgttcttcggggcgaaaactctcaaggatcttaccgctgttgagatccagttcgatgtaacccactcgtgcacccaactgatcttcagcatcttttactttcaccagcgtttctgggtgagcaaaaacaggaaggcaaaatgccgcaaaaaagggaataagggcgacacggaaatgttgaatactcatactcttcctttttcaatattattgaagcatttatcagggttattgtctcatgagcggatacatatttgaatgtatttagaaaaataaacaaataggggttccgcgcacatttccccgaaaagtgccacctgacgtc

SEQ ID NO: 47 - DNA, 8143 bp, Artificial Sequence
  HEK293T AAT Vector
aaaggcggccgccaccatggggaccctcagcgctccgccttgtacccagaggattaagtggaaagggctgctgctgacagccagcctgttaaacttctggaacttgcccaccaccgctgaggacccacaaggcgacgcggcccagaagaccgatacaagccaccacgaccaagatcatcctaccttcaacaagatcactcccaacctcgctgagtttgccttctccttgtatcgccagcttgcgcaccaatccaattcaaccaatatattcttcagcccagtaagtatcgctactgcgtttgcaatgcttagtttgggaacaaaagcggacactcacgacgaaatccttgagggcttgaatttcaacttgaccgaaattccggaggcccagattcacgaagggttccaggagcttttgaggacactgaaccagccagactcacaattgcaacttacaaccggcaacggactgtttctttccgagggccttaaacttgttgataaatttcttgaagacgtcaagaagctgtaccactcagaagcatttacagtcaacttcggcgataccgaagaggcaaagaagcaaatcaacgactatgtggagaagggaactcaggggaaaatagtagacctggtaaaggaattggaccgcgacacggtattcgcgttggttaattacatctttttcaagggtaagtgggaacggccatttgaagtgaaggacaccgaagaagaagacttccacgtagaccaggtaactactgttaaagtcccaatgatgaaacgattgggtatgtttaacattcagcattgtaagaagctctcatcctgggttcttttgatgaaatacttggggaatgcaacggccatattctttcttccggatgagggaaagttgcaacacctggaaaatgaactcacacacgacatcattacgaaattcttggaaaatgaagaccggaggtccgcttctttgcacctgccaaaactcagtataacgggtacatatgacctcaagtccgtcctcggtcaactgggaataactaaggtcttttctaacggagcagatttgagcggcgtcacagaagaagcacctttgaaacttagtaaggctgtccataaagcggtactcacaattgacgagaaagggaccgaagctgcgggggctatgtttctggaggcaatcccaatgagcataccaccagaagttaaatttaacaaacctttcgttttcctcatgatagagcaaaacacaaaaagtccgctgtttatgggaaaggtagtgaatcctacccagaaagggagcgctagcgaaaacctgtacttccaaggcacttccgcttggtcccatcctcagtttgagaaaggcggaggtagtggcggaggatccggtggatctgcttggagccatccacagttcgaaaagggatcccaccatcatcaccatcaccaccaccatcattaatgactgagtagtctagaagttgtctcctcctgcactgactgactgatacaatcgatttctggatccgcaggcctaatcaacctctggattacaaaatttgtgaaagattgactggtattcttaactatgttgctccttttacgctatgtggatacgctgctttaatgcctttgtatcatgctattgcttcccgtatggctttcattttctcctccttgtataaatcctggttgctgtctctttatgaggagttgtggcccgttgtcaggcaacgtggcgtggtgtgcactgtgtttgctgacgcaacccccactggttggggcattgccaccacctgtcagctcctttccgggactttcgctttccccctccctattgccacggcggaactcatcgccgcctgccttgcccgctgctggacaggggctcggctgttgggcactgacaattccgtggtgttgtcggggaagctgacgtcctttccatggctgctcgcctgtgttgccacctggattctgcgcgggacgtccttctgctacgtcccttcggccctcaatccagcggaccttccttcccgcggcctgctgccggctctgcggcctcttccgcgtcttcgccttcgccctcagacgagtcggatctccctttgggccgcctccccgcctgtctagcttgactgactgagatacagcgtaccttcagctcacagacatgataagatacattgatgagtttggacaaaccacaactagaatgcagtgaaaaaaatgctttatttgtgaaatttgtgatgctattgctttatttgtaaccattataagctgcaataaacaagttaacaacaacaattgcattcattttatgtttcaggttcagggggaggtgtgggaggttttttaaagcaagtaaaacctctacaaatgtggtattggcccatctctatcggtatcgtagcataaccccttggggcctctaaacgggtcttgaggggttttttgtgcccctcgggccggattgctatctaccggcattggcgcagaaaaaaatgcctgatgcgacgctgcgcgtcttatactcccacatatgccagattcagcaacggatacggcttccccaacttgcccacttccatacgtgtcctccttaccagaaatttatccttaaggtcgtcagctatcctgcaggcgatctctcgatttcgatcaagacattcctttaatggtcttttctggacaccactaggggtcagaagtagttcatcaaactttcttccctccctaatctcattggttaccttgggctatcgaaacttaattaagcgatctgcatctcaattagtcagcaaccatagtcccgcccctaactccgcccatcccgcccctaactccgcccagttccgcccattctccgccccatcgctgactaattttttttatttatgcagaggccgaggccgcctcggcctctgagctattccagaagtagtgaggaggcttttttggaggcctaggcttttgcaaaggaggtagccaacatgattgaacaagatggattgcacgcaggttctcccgccgcttgggtggagaggctattcggctatgactgggcacaacagacaatcggctgctctgatgccgccgtgttccggctgtcagcgcaggggcgcccggttctttttgtcaagaccgacctgtccggtgccctgaatgaactccaggacgaggcagcgcggctatcgtggctggccacgacgggcgttccttgcgcagctgtgctcgacgttgtcactgaagcgggaagggactggctgctattgggcgaagtgccggggcaggatctcctgtcatctcaccttgctcctgccgagaaagtatccatcatggctgatgcaatgcggcggctgcatacgcttgatccggctacctgcccattcgaccaccaagcgaaacatcgcatcgagcgagcacgtactcggatggaagccggtcttgtcgatcaggatgatctggacgaagagcatcaggggctcgcgccagccgaactgttcgccaggctcaaggcgcggatgcccgacggcgaggatctcgtcgtgacccacggcgatgcctgcttgccgaatatcatggtggaaaatggccgcttttctggattcatcgactgtggccggctgggtgtggcggaccgctatcaggacatagcgttggctacccgtgatattgctgaagagcttggcggcgaatgggctgaccgcttcctcgtgctttacggtatcgccgctcccgattcgcagcgcatcgccttctatcgccttcttgacgagttcttctagtatgtaagccctgtgccttctagttgccagccatctgttgtttgcccctcccccgtgccttccttgaccctggaaggtgccactcccactgtcctttcctaataaaatgaggaaattgcatcgcattgtctgagtaggtgtcattctattctggggggtggggtggggcaggacagcaagggggaggattgggaagacaatagcaggcatgctggggatgcggtgggctctatggttaattaaccagtcaagtcagctacttggcgagatcgacttgtctgggtttcgactacgctcagaattgcgtcagtcaagttcgatctggtccttgctattgcacccgttctccgattacgagtttcatttaaatcatgtgagcaaaaggccagcaaaaggccaggaaccgtaaaaaggccgcgttgctggcgtttttccataggctccgcccccctgacgagcatcacaaaaatcgacgctcaagtcagaggtggcgaaacccgacaggactataaagataccaggcgtttccccctggaagctccctcgtgcgctctcctgttccgaccctgccgcttaccggatacctgtccgcctttctcccttcgggaagcgtggcgctttctcatagctcacgctgtaggtatctcagttcggtgtaggtcgttcgctccaagctgggctgtgtgcacgaaccccccgttcagcccgaccgctgcgccttatccggtaactatcgtcttgagtccaacccggtaagacacgacttatcgccactggcagcagccactggtaacaggattagcagagcgaggtatgtaggcggtgctacagagttcttgaagtggtggcctaactacggctacactagaagaacagtatttggtatctgcgctctgctgaagccagttaccttcggaaaaagagttggtagctcttgatccggcaaacaaaccaccgctggtagcggtggtttttttgtttgcaagcagcagattacgcgcagaaaaaaaggatctcaagaagatcctttgatcttttctacggggtctgacgctcagtggaacgaaaactcacgttaagggattttggtcatgagattatcaaaaaggatcttcacctagatccttttaaattaaaaatgaagttttaaatcaatctaaagtatatatgagtaaacttggtctgacagttaccaatgcttaatcagtgaggcacctatctcagcgatctgtctatttcgttcatccatagttgcatttaaatttccgaactctccaaggccctcgtcggaaaatcttcaaacctttcgtccgatccatcttgcaggctacctctcgaacgaactatcgcaagtctcttggccggccttgcgccttggctattgcttggcagcgcctatcgccaggtattactccaatcccgaatatccgagatcgggatcacccgagagaagttcaacctacatcctcaatcccgatctatccgagatccgaggaatatcgaaatcggggcgcgcctggtgtaccgagaacgatcctctcagtgcgagtctcgacgatccatatcgttgcttggcagtcagccagtcggaatccagcttgggacccaggaagtccaatcgtcagatattgtactcaagcctggtcacggcagcgtaccgatctgtttaaacctagatattgatagtctgatcggtcaacgtataatcgagtcctagcttttgcaaacatctatcaagagacaggatcagcaggaggctttcgcatgagtattcaacatttccgtgtcgcccttattcccttttttgcggcattttgccttcctgtttttgctcacccagaaacgctggtgaaagtaaaagatgctgaagatcagttgggtgcgcgagtgggttacatcgaactggatctcaacagcggtaagatccttgagagttttcgccccgaagaacgctttccaatgatgagcacttttaaagttctgctatgtggcgcggtattatcccgtattgacgccgggcaagagcaactcggtcgccgcatacactattctcagaatgacttggttgagtattcaccagtcacagaaaagcatcttacggatggcatgacagtaagagaattatgcagtgctgccataaccatgagtgataacactgcggccaacttacttctgacaacgattggaggaccgaaggagctaaccgcttttttgcacaacatgggggatcatgtaactcgccttgatcgttgggaaccggagctgaatgaagccataccaaacgacgagcgtgacaccacgatgcctgtagcaatggcaacaaccttgcgtaaactattaactggcgaactacttactctagcttcccggcaacagttgatagactggatggaggcggataaagttgcaggaccacttctgcgctcggcccttccggctggctggtttattgctgataaatctggagccggtgagcgtgggtctcgcggtatcattgcagcactggggccagatggtaagccctcccgtatcgtagttatctacacgacggggagtcaggcaactatggatgaacgaaatagacagatcgctgagataggtgcctcactgattaagcattggtaaccgattctaggtgcattggcgcagaaaaaaatgcctgatgcgacgctgcgcgtcttatactcccacatatgccagattcagcaacggatacggcttccccaacttgcccacttccatacgtgtcctccttaccagaaatttatccttaagatcgtttaaactcgactctggctctatcgaatctccgtcgtttcgagcttacgcgaacagccgtggcgctcatttgctcgtcgggcatcgaatctcgtcagctatcgtcagcttacctttttggcagcgatcgcggctcccgacatcttggaccattagctccacaggtatcttcttccctctagtggtcataacagcagcttcagctacctctcaattcaaaaaacccctcaagacccgtttagaggccccaaggggttatgctatcaatcgttgcgttacacacacaaaaaaccaacacacatccatcttcgatggatagcgattttattatctaactgctgatcgagtgtagccagatctagtaatcaattacggggtcattagttcatagcccatatatggagttccgcgttacataacttacggtaaatggcccgcctggctgaccgcccaacgacccccgcccattgacgtcaataatgacgtatgttcccatagtaacgccaatagggactttccattgacgtcaatgggtggagtatttacggtaaactgcccacttggcagtacatcaagtgtatcatatgccaagtacgccccctattgacgtcaatgacggtaaatggcccgcctggcattatgcccagtacatgaccttatgggactttcctacttggcagtacatctacgtattagtcatcgctattaccatgctgatgcggttttggcagtacatcaatgggcgtggatagcggtttgactcacggggatttccaagtctccaccccattgacgtcaatgggagtttgttttggcaccaaaatcaacgggactttccaaaatgtcgtaacaactccgccccattgacgcaaatgggcggtaggcgtgtacggtgggaggtctatataagcagagctggtttagtgaaccgtcagatcgcctggagacgccatccacgctgttttgacctccatagaagacaccgggaccgatccagcctcccctcgaagcttacatgtggtaccgagctcggatcctgagaacttcagggtgagtctatgggacccttgatgttttctttccccttcttttctatggttaagttcatgtcataggaaggggagaagtaacagggtacacatattgaccaaatcagggtaattttgcatttgtaattttaaaaaatgctttcttcttttaatatacttttttgtttatcttatttctaatactttccctaatctctttctttcagggcaataatgatacaatgtatcatgcctctttgcaccattctaaagaataacagtgataatttctgggttaaggcaatagcaatatttctgcatataaatatttctgcatataaattgtaactgatgtaagaggtttcatattgctaatagcagctacaatccagctaccattctgcttttattttatggttgggataaggctggattattctgagtccaagctaggcccttttgctaatcatgttcatacctcttatcttcctcccacagctcctgggcaacgtgctggtctgtgtgctggcccatcactttggc